European Patent Specification EP 3 856 910 B1, published November 20, 2024. Title: EXPRESSION VECTORS FOR EUKARYOTIC EXPRESSION SYSTEMS. Applicant: Merck Sharp & Dohme Corp. Du, Zhimei Jiang, Bo Tang, Xiaoyan. The sequence listing filed with the application follows.

SEQUENCE LISTING (29 sequences)

SEQ ID NO: 1 - DNA, 569 bp, Artificial Sequence
  IRES-1
cccctaacgttactggccgaagccgcttggaataaggccggtgtgcgtttgtctatatgttattttccaccatattgccgtcttttggcaatgtgagggcccggaaacctggccctgtcttcttgacgagcattcctaggggtctttcccctctcgccaaaggaatgcaaggtctgttgaatgtcgtgaaggaagcagttcctctggaagcttcttgaagacaaacaacgtctgtagcgaccctttgcaggcagcggaaccccccacctggcgacaggtgcctctgcggccaaaagccacgtgtataagatacacctgcaaaggcggcacaaccccagtgccacgttgtgagttggatagttgtggaaagagtcaaatggctctcctcaagcgtattcaacaaggggctgaaggatgcccagaaggtaccccattgtatgggatctgatctggggcctcggtgcacatgctttacatgtgtttagtcgaggttaaaaaacgtctaggccccccgaaccacggggacgtggttttcctttgaaaaacacgatgataatatggccacaacc

SEQ ID NO: 2 - DNA, 556 bp, Artificial Sequence
  IRES-2
cccctaacgttactggccgaagccgcttggaataaggccggtgtgcgtttgtctatatgttattttccaccatattgccgtcttttggcaatgtgagggcccggaaacctggccctgtcttcttgacgagcattcctaggggtctttcccctctcgccaaaggaatgcaaggtctgttgaatgtcgtgaaggaagcagttcctctggaagcttcttgaagacaaacaacgtctgtagcgaccctttgcaggcagcggaaccccccacctggcgacaggtgcctctgcggccaaaagccacgtgtataagatacacctgcaaaggcggcacaaccccagtgccacgttgtgagttggatagttgtggaaagagtcaaatggctctcctcaagcgtattcaacaaggggctgaaggatgcccagaaggtaccccattgtatgggatctgatctggggcctcggtgcacatgctttacatgtgtttagtcgaggttaaaaaacgtctaggccccccgaaccacggggacgtggttttcctttgaaaaacacgatgataa

SEQ ID NO: 3 - DNA, 549 bp, Artificial Sequence
  IRES-3
cccctaacgttactggccgaagccgcttggaataaggccggtgtgcgtttgtctatatgttattttccaccatattgccgtcttttggcaatgtgagggcccggaaacctggccctgtcttcttgacgagcattcctaggggtctttcccctctcgccaaaggaatgcaaggtctgttgaatgtcgtgaaggaagcagttcctctggaagcttcttgaagacaaacaacgtctgtagcgaccctttgcaggcagcggaaccccccacctggcgacaggtgcctctgcggccaaaagccacgtgtataagatacacctgcaaaggcggcacaaccccagtgccacgttgtgagttggatagttgtggaaagagtcaaatggctctcctcaagcgtattcaacaaggggctgaaggatgcccagaaggtaccccattgtatgggatctgatctggggcctcggtgcacatgctttacatgtgtttagtcgaggttaaaaaacgtctaggccccccgaaccacggggacgtggttttcctttgaaaaacacg

SEQ ID NO: 4 - DNA, 6215 bp, Artificial Sequence
  pCLD116
ccaatgatcttaagttaaccctagaaagataatcatattgtgacgtacgttaaagataatcatgcgtaaaattgacgcatgtgttttatcggtctgtatatcgaggtttatttattaatttgaatagatattaagttttattatatttacacttacatactaataataaattcaacaaacaatttatttatgtttatttatttattaaaaaaaaacaaaaactcaaaatttcttctataaagtaacaaaacttttatcgaatttgcagcccgggactagctagagggacagcccccccccaaagcccccagggatgtaattacgtccctcccccgctagggggcagcagcgagccgcccggggctccgctccggtccggcgctccccccgcatccccgagccggcagcgtgcggggacagcccgggcacggggaaggtggcacgggatcgctttcctctgaacgcttctcgctgctctttgagcctgcagacacctggggggatacggggaaaacttaagatccgaccggtgctgtggaatgtgtgtcagttagggtgtggaaagtccccaggctccccagcaggcagaagtatgcaaagcatgcatctcaattagtcagcaaccaggtgtggaaagtccccaggctccccagcaggcagaagtatgcaaagcatgcatctcaattagtcagcaaccatagtcccgcccctaactccgcccatcccgcccctaactccgcccagttccgcccattctccgctccatcgttcagattttaccacatttgtagaggttttacttgctttaaaaaacctcccacacctccccctgaacctgaaacataaaatgaatgcaattgttgttgttaacttgtttattgcagcttataatggttacaaataaagcaatagcatcacaaatttcacaaataaagcatttttttcactgcattctagttgtggtttgtccaaactcatcaatgtatcttatcatgtctgctcgaagcggccggccgccccgactctagattagtttttgtattggaagggctcgtcgccagtctcattgagaaggcatgtgcggacgatggcttctgtcactgcaaaggggtcacaattggcagaggggcggcggtcttcaaagtaacctttcttctcctggccgacagtccggggaatgcggatgctggcactgcgattggcgacaccagcagaaaagtcgttgatgttggacgtttcgtggaacccagtcagacgacgggcattgtccaggccccccttgggatcgtaggctcgaatgtggtaccggtgccgcttgcttagtttctcgatggcctcctcgatgtgcttcagaccattctcctcccgcatggccttggtgctaaagttggtatggcagcctgcaccattccagttcccaggaatgggcttggggtcaaaggttgctattaccccaaagtcttcacatactcgatgcaagatgaaacgggccacccagagatgatctcccatgcggattccttcacagggtcctatttggaactcccactgggcaggcatgacctcagcatttgttcctgtaatcttgaccccagcatacaagcaggcgcggtagtgagcctccacgatatccctgccataggctttgtctgcgcccacaccacagtaatacggaccttggggcccaggaaagccattggaaggccaaccaaaagggtgcccatctgttcccatcagagtatactcctgttccattccaaaccaggggtgctggttgctcaccatgtccattatccgtttacacgagtgccttaaattggtctctgcaggcttccggttgtacttgaaaacttcacagaacaccagcttgttgggatctctgcggaaggggtcccgaaacatggcaacagggctgagatacatgtcactgttggagccctcagactgaaaggtactagagccatcaaaattccactcaggtaactcttctacacacttgggctcacagtccagggtgcgggttttgcagcgcagtccttctccagtaccatcaacccagatatacatggcttggactttctcaccctggggcaggcacaagtacatttgcttgatgtttttgttcaagtgggaacttgctgaggtggccatggtggcggctttgcaaaagcctaggcctccaaaaaagcctcctcactacttctggaatagctcagaggccgaggcggcctcggcctctgcataaataaaaaaaattagtcagcgatggggcggagaatgggcggaactgggcggagttaggggcgggatgggcggagttaggggcgggactatggttgctgactaattgagatgcaatcactgacacacattccacagctgcctcgcgcgtttcggtgatgacggtgaaaacctctgacacatgcagctcccggagacggtcacagcttgtctgtaagcggatgccgggagcagacaagcccgtcagggcgcgtcagcgggtgttggcgggtgtcggggcgcagccatgacccagtcacgtagcgatagcggagtgtatactggcttaactatgcggcatcagagcagattgtactgagcctcgagcgatgtacgggccagatatacgcgttgacattgattattgactagttattaatagtaatcaattacggggtcattagttcatagcccatatatggagttccgcgttacataacttacggtaaatggcccgcctggctgaccgcccaacgacccccgcccattgacgtcaataatgacgtatgttcccatagtaacgccaatagggactttccattgacgtcaatgggtggactatttacggtaaactgcccacttggcagtacatcaagtgtatcatatgccaagtacgccccctattgacgtcaatgacggtaaatggcccgcctggcattatgcccagtacatgaccttatgggactttcctacttggcagtacatctacgtattagtcatcgctattaccatggtgatgcggttttggcagtacatcaatgggcgtggatagcggtttgactcacggggatttccaagtctccaccccattgacgtcaatgggagtttgttttggcaccaaaatcaacgggactttccaaaatgtcgtaacaactccgccccattgacgcaaatgggcggtaggcgtgtacggtgggaggtctatataagcagagctctctggctaactagagaacccactgcttactggcttatcgaaattaatacgactcactatagcaattgcacgtgtggccacaggtaagtttaaagctcaggtcgagaccgggcctttgtccggcgctcccttggagcctacctagactcagccggctctccacgctttgcctgaccctgcttgctcaactctacgtctttgtttcgttttctgttcctttctctccacaggcggatccgaattctgaagatctagatccccctcgctttcttgctgtccaatttctattaaaggttcctttgttccctaagtccaactactaaactgggggatattatgaagggccttgagcatctggattctgcctaataaaaaacatttattttcattgcaatgatgtatttaaattatttctgaatattttactaaaaagggaatgtgggaggtcagtgcatttaaaacataaagaaatgaagagggggatcttcgcgaatccatcgatgagggacagcccccccccaaagcccccagggatgtaattacgtccctcccccgctagggggcagcagcgagccgcccggggctccgctccggtccggcgctccccccgcatccccgagccggcagcgtgcggggacagcccgggcacggggaaggtggcacgggatcgctttcctctgaacgcttctcgctgctctttgagcctgcagacacctggggggatacggggaaaatagacaccgcggtggagctccagcttttgttccctttagtgagggttaattagttcttaatacgactcactatagggcgaattggctaccgggccgcccatcgagggtatcataagcttatatctataacaagaaaatatatatataataagttatcacgtaagtagaacatgaaataacaatataattatcgtatgagttaaatcttaaaagtcacgtaaaagataatcatgcgtcattttgactcacgcggtcgttatagttcaaaatcagtgacacttaccgcattgacaagcacgcctcacgggagctccaagcggcgactgagatgtcctaaatgcacagcgacggattcgcgctatttagaaagagagagcaatatttcaagaatgcatgcgtcaattttacgcagactatctttctagggttaaatcgatatcggaaagaacatgtgagcaaaaggccagcaaaaggccaggaaccgtaaaaaggccgcgttgctggcgtttttccataggctccgcccccctgacgagcatcacaaaaatcgacgctcaagtcagaggtggcgaaacccgacaggactataaagataccaggcgtttccccctggaagctccctcgtgcgctctcctgttccgaccctgccgcttaccggatacctgtccgcctttctcccttcgggaagcgtggcgctttctcatagctcacgctgtaggtatctcagttcggtgtaggtcgttcgctccaagctgggctgtgtgcacgaaccccccgttcagcccgaccgctgcgccttatccggtaactatcgtcttgagtccaacccggtaagacacgacttatcgccactggcagcagccactggtaacaggattagcagagcgaggtatgtaggcggtgctacagagttcttgaagtggtggcctaactacggctacactagaagaacagtatttggtatctgcgctctgctgaagccagttaccttcggaaaaagagttggtagctcttgatccggcaaacaaaccaccgctggtagcggtggtttttttgtttgcaagcagcagattacgcgcagaaaaaaaggatctcaagaagatcctttgatcttttctacggggtctgacgctcagtggaacgaaaactcacgttaagggattttggtcatgagattatcaaaaaggatcttcacctagatccttttaaattaaaaatgaagttttaaatcaatctaaagtatatatgagtaaacttggtctgacagttaccaatgcttaatcagtgaggcacctatctcagcgatctgtctatttcgttcatccatagttgcctgactccccgtcgtgtagataactacgatacgggagggcttaccatctggccccagtgctgcaatgataccgcgagacccacgctcaccggctccagatttatcagcaataaaccagccagccggaagggccgagcgcagaagtggtcctgcaactttatccgcctccatccagtctattaattgttgccgggaagctagagtaagtagttcgccagttaatagtttgcgcaacgttgttgccattgctacaggcatcgtggtgtcacgctcgtcgtttggtatggcttcattcagctccggttcccaacgatcaaggcgagttacatgatcccccatgttgtgcaaaaaagcggttagctccttcggtcctccgatcgttgtcagaagtaagttggccgcagtgttatcactcatggttatggcagcactgcataattctcttactgtcatgccatccgtaagatgcttttctgtgactggtgagtactcaaccaagtcattctgagaatagtgtatgcggcgaccgagttgctcttgcccggcgtcaatacgggataataccgcgccacatagcagaactttaaaagtgctcatcattggaaaacgttcttcggggcgaaaactctcaaggatcttaccgctgttgagatccagttcgatgtaacccactcgtgcacccaactgatcttcagcatcttttactttcaccagcgtttctgggtgagcaaaaacaggaaggcaaaatgccgcaaaaaagggaataagggcgacacggaaatgttgaatactcatactcttcctttttcaatattattgaagcatttatcagggttattgtctcatgagcggatacatatttgaatgtatttagaaaaataaacaaataggggttccgcgcacatttccccgaaaagtgccacctgacgtc

SEQ ID NO: 5 - DNA, 9542 bp, Artificial Sequence
  pCLD21
ccttcccttctaccacaccctaattgtaatccattttaatttcctggtcacagtcctgtctctccttccattgtaccttgcccttttctaaagagcgactgcaaagtatgtttgcgtaggtgaggatctaaaactttatgaggtacgaacatcacagaattactttgtaatttcagtttattgtaggcttggctttttggggagggtttacgtcttagacctcttagtgcttctttgtttcatggtgttctaacttcgaagcatctctgtagctttaatggattccttttctgaaagctttgctctctttcttccccctcggctttctcttaggcaagagggctaactgtaaagtaaggcttactgccttgtgtttccaaatgtgtccgaagaggaagtgtcttctgtgaatcctgttatgcatgaataacaggaaatagaaagaaattcactttcattattataaaagtaatatgttcgtttaaaaaattctaatgaagagctggagatgcaacccaggggtagagcacacactcagcatgcaggaggccctgggtccaatcttggaatctcctctcagttaacctgatctctagctgattagtagtgagtgcaagcccactttcctcttctgcctcattgctcagtgataacagctgttaaactttgtcttattctaaaactacctctgtgcaaatgctagcacaataatatatatcatatgcacatgattttttttttatcttgaaaagtaagtcagtatagctacaaagttcacttggcattgtcaacatttcacaggcgtaatattcctcctctagtactgtcctcttcattctttgtgaccaagtttggagagagtgcacaaatgccagggaggtttgtgggaaggtttctcatgttctggtaaggcgagtaagaaaatagtctcatgcaggtgaaatgagtgctatgcagtatatattataccagagaacagcaaatgaccaaattcacactgaactagttcagtaaaattggctttgtcaaagctttccttgcttaaaatgtaattccctgtcatcctagttctggtctggattcttttcctggagtcttgacttccagattccctgtggacttttgtttgagtttcaagcttttgaaatatagaaacctatctaacttaacaaacttgggagagaaaagactccagaacaactgaaaacagaccaggctaaatgaatagactttattcctctcttcttacctgcagttttcagatatgcagagttggagcggatcttagaggttgattcattcatgcctgaagaaaacacattttatagaccctgtgcccaagttcgtggtggacatcaccctttatttactaattgcactacataacaggcattttagaagactgctccagtcagagaccccgccttagaggaatctgtaaaccctgaactcctatcactcatgagcactagttatgtttggaatgccgtattaaaacaaaagttacatttctaaacttaaaattttctagcacagagacagtgggagtagctaactttgatagacatttttctactaaaagtctttctaagtacataatcttctgtaagttggaaaacagcaaaatagaacgtctcctacgtagttaatctttttgcataatttgcacatgtaggagttattagtatacgggtaagttttcactttttcccccaactggagtgtcttgtggctgggtttgaaaaagggaacgggaggccgctggaggggattggtaaatgagataaaacaccactcattcaactcagtgactcagcatttaaattttccataaaaggattaaaggaaaattaaacaaattcttaaagccaagactctggagaaacttgttggtgtgctttagttttcactgttatgactcatgaatttatgcataaattagtacatttataaaaacatagcctttttagagttttctgtttggctaaagtgccattgttagcatttggaattacctttttatgtcttatattttttccaaataaaaataaatgtttctgctgtcttactactgaaactacgttgtgagcactttaaatttctcaaagcagtttcgcctgttatacttggcgcttagtcatcgtcgtacacaacaggacctgattaagaaggctgtgctgcctctaagccgggctagattgtagccactagcaaccaggctgcaataatttccctttgatgacatcatccactgtggaagaacccagttgcttcagccagtcgaactatacagttccaacctcatcaaatatggcatctcccttgcctgctatagcagggggaggaaaaaatgccaccatctttttaatctagcaagcttctcttttcttcatctttttttttttcttttaaaaaaattctgatcatggatgcttcttccgatccctatttgccttatgacgggggaggagacaatatccccttgagggaattacataaaagaggtaagagcatccccttgctctgaatcctctgttggttgttgtgcatgcggctgggcggttctggggacaggctgtctgttgtcctcttgctgcaatgtgctgcttagttgccctgccttgttgctgtgggagaatgcgaccttcccagcagggctggccctccctgattgtttgctctgtgcagattagccctgcttcagatcacatagggctgcagactccatcttctgtgtgaaaatgctttcggtttgattgcagaaataagctgcctttacagccagctaaagtcctggtggttggttggcacctgcaaagtagtatttttgtacctctggaaacttatattttctttacacagcaatatcaagtgccggtatgccattctgttttggctgctgccaattaccatgtagactttgcaccacagagtaatagtaaaagctcctagctgcattttataacatttaaaaatagcaggaaagaagaattatttttgatttaacatgtttttgtcatttaacgtcttaactgattgacatactatattgtctgtctcgtgggtatcttgtacaacttgataggataaagcaatttagtttttttttttttttttaaatacatccagaatgtaagtcgtcagtagttttcgaacagataagtaatggtgttaatcttttggcaggctttgccttggtctccttaaagctaattaggtgttacttaattaaactgctcttttgctcattttcttaaattatttttttaaaagatagttggcatttgctgttctagaaataaacttcaagaaacattctttagccagatgacttcatgtatgagccatgttagtttgaattatttgcttggtgttataaactttatggtttaataccaacttttattatgtttacaaggtaaataaggaaaatttcaagtacattttgtatcctgagaacaaatttaagttccatagaatttaggaattacaatgtattcaacagatacttacttgtcatactgtgcctgcaaaacaataattagactctgaacaggtgcaacaattttctgtagaattagacaagtcttcttttggcaggtgttactaagtaggccatttcccaaggaacagggaatttgccaggcttttgtggtggagagaatagaatgaataaatgctgtggggagtaaagagcttgtcagaagatgattagttctgtggcaccaaaaccaagagatcagttttcctgtgagaagtaaaggaagcattgtagaaaaatagatgtgttgaagtctaccggtggagttccgcgttacataacttacggtaaatggcccgcctggctgaccgcccaacgacccccgcccattgacgtcaataatgacgtatgttcccatagtaacgccaatagggactttccattgacgtcaatgggtggagtatttacggtaaactgcccacttggcagtacatcaagtgtatcatatgccaagtacgccccctattgacgtcaatgacggtaaatggcccgcctggcattatgcccagtacatgaccttatgggactttcctacttggcagtacatctacgtattagtcatcgctattaccattgtgatgcggttttggcagtacatcaatgggcgtggatagcggtttgactcacggggatttccaagtctccaccccattgacgtcaatgggagtttgttttggcaccaaaatcaacgggactttccaaaatgtcgtaacaactccgccccattgacgcaaatgggcggtaggcgtgtacggtgggaggtctatataagcagagctcgtttagtgaaccgtcagatctacctcttccgcatcgctgtctgcgagggccagctgttggggtgagtactccctctcaaaagcgggcatgacttctgcgctaagattgtcagtttccaaaaacgaggaggatttgatattcacctggcccgcggtgatgcctttgagggtggccgcgtccatctggtcagaaaagacaatctttttgttgtcaagcttccttgatgatgtcatacttatcctgtcccttttttttccacagctcgcggttgaggacaaactcttcgcggtctttccagtactcttggatcggaaacccgtcggcctccgaacggtactccgccaccgagggacctgagcgagtccgcatcgaccggatcggaaaacctcggatccgaattcatagataactgatccagtgcccctaacgttactggccgaagccgcttggaataaggccggtgtgcgtttgtctatatgttattttccaccatattgccgtcttttggcaatgtgagggcccggaaacctggccctgtcttcttgacgagcattcctaggggtctttcccctctcgccaaaggaatgcaaggtctgttgaatgtcgtgaaggaagcagttcctctggaagcttcttgaagacaaacaacgtctgtagcgaccctttgcaggcagcggaaccccccacctggcgacaggtgcctctgcggccaaaagccacgtgtataagatacacctgcaaaggcggcacaaccccagtgccacgttgtgagttggatagttgtggaaagagtcaaatggctctcctcaagcgtattcaacaaggggctgaaggatgcccagaaggtaccccattgtatgggatctgatctggggcctcggtgcacatgctttacatgtgtttagtcgaggttaaaaaacgtctaggccccccgaaccacggggacgtggttttcctttgaaaaacacgatgataatatggccacaaccatggccacctcagcaagttcccacttgaacaaaaacatcaagcaaatgtacttgtgcctgccccagggtgagaaagtccaagccatgtatatctgggttgatggtactggagaaggactgcgctgcaaaacccgcaccctggactgtgagcccaagtgtgtagaagagttacctgagtggaattttgatggctctagtacctttcagtctgagggctccaacagtgacatgtatctcagccctgttgccatgtttcgggaccccttccgcagagatcccaacaagctggtgttctgtgaagttttcaagtacaaccggaagcctgcagagaccaatttaaggcactcgtgtaaacggataatggacatggtgagcaaccagcacccctggtttggaatggaacaggagtatactctgatgggaacagatgggcacccttttggttggccttccaatggctttcctgggccccaaggtccgtattactgtggtgtgggcgcagacaaagcctatggcagggatatcgtggaggctcactaccgcgcctgcttgtatgctggggtcaagattacaggaacaaatgctgaggtcatgcctgcccagtgggagttccaaataggaccctgtgaaggaatccgcatgggagatcatctctgggtggcccgtttcatcttgcatcgagtatgtgaagactttggggtaatagcaacctttgaccccaagcccattcctgggaactggaatggtgcaggctgccataccaactttagcaccaaggccatgcgggaggagaatggtctgaagcacatcgaggaggccatcgagaaactaagcaagcggcaccggtaccacattcgagcctacgatcccaaggggggcctggacaatgcccgtcgtctgactgggttccacgaaacgtccaacatcaacgacttttctgctggtgtcgccaatcgcagtgccagcatccgcattccccggactgtcggccaggagaagaaaggttactttgaagaccgccgcccctctgccaattgtgacccctttgcagtgacagaagccatcgtccgcacatgccttctcaatgagactggcgacgagcccttccaatacaaaaactaatctagatccccctcgctttcttgctgtccaatttctattaaaggttcctttgttccctaagtccaactactaaactgggggatattatgaagggccttgagcatctggattctgcctaataaaaaacatttattttcattgcaatgatgtatttaaattatttctgaatattttactaaaaagggaatgtgggaggtcagtgcatttaaaacataaagaaatgaagagggggatcttcgcgacctgcaggtctccctatagtgagtcgtattaatttcgataagccagctgcattaatgaatcggccaacgcgcggggagaggcggtttgcgtattgggcgctcttccgcttcctcgctcactgactcgctgcgctcggtcgttcggctgcggcgagcggtatcagctcactcaaaggcggtaatacggttatccacagaatcaggggataacgcaggaaagaacatgtgagcaaaaggccagcaaaaggccaggaaccgtaaaaaggccgcgttgctggcgtttttccataggctccgcccccctgacgagcatcacaaaaatcgacgctcaagtcagaggtggcgaaacccgacaggactataaagataccaggcgtttccccctggaagctccctcgtgcgctctcctgttccgaccctgccgcttaccggatacctgtccgcctttctcccttcgggaagcgtggcgctttctcatagctcacgctgtaggtatctcagttcggtgtaggtcgttcgctccaagctgggctgtgtgcacgaaccccccgttcagcccgaccgctgcgccttatccggtaactatcgtcttgagtccaacccggtaagacacgacttatcgccactggcagcagccactggtaacaggattagcagagcgaggtatgtaggcggtgctacagagttcttgaagtggtggcctaactacggctacactagaaggacagtatttggtatctgcgctctgctgaagccagttaccttcggaaaaagagttggtagctcttgatccggcaaacaaaccaccgctggtagcggtggtttttttgtttgcaagcagcagattacgcgcagaaaaaaaggatctcaagaagatcctttgatcttttctacggggtctgacgctcagtggaacgaaaactcacgttaagggattttggtcatgagattatcaaaaaggatcttcacctagatccttttaaattaaaaatgaagttttaaatcaatctaaagtatatatgagtaaacttggtctgacagttaccaatgcttaatcagtgaggcacctatctcagcgatctgtctatttcgttcatccatagttgcctgactccccgtcgtgtagataactacgatacgggagggcttaccatctggccccagtgctgcaatgataccgcgagacccacgctcaccggctccagatttatcagcaataaaccagccagccggaagggccgagcgcagaagtggtcctgcaactttatccgcctccatccagtctattaattgttgccgggaagctagagtaagtagttcgccagttaatagtttgcgcaacgttgttgccattgctacaggcatcgtggtgtcacgctcgtcgtttggtatggcttcattcagctccggttcccaacgatcaaggcgagttacatgatcccccatgttgtgcaaaaaagcggttagctccttcggtcctccgatcgttgtcagaagtaagttggccgcagtgttatcactcatggttatggcagcactgcataattctcttactgtcatgccatccgtaagatgcttttctgtgactggtgagtactcaaccaagtcattctgagaatagtgtatgcggcgaccgagttgctcttgcccggcgtcaatacgggataataccgcgccacatagcagaactttaaaagtgctcatcattggaaaacgttcttcggggcgaaaactctcaaggatcttaccgctgttgagatccagttcgatgtaacccactcgtgcacccaactgatcttcagcatcttttactttcaccagcgtttctgggtgagcaaaaacaggaaggcaaaatgccgcaaaaaagggaataagggcgacacggaaatgttgaatactcatactcttcctttttcaatattattgaagcatttatcagggttattgtctcatgagcggatacatatttgaatgtatttagaaaaataaacaaataggggttccgcgcacatttccccgaaaagtgccacctgacgtctaagaaaccattattatcatgacattaacctataaaaataggcgtatcacgaggccctttcgtctcgcgcgtttcggtgatgacggtgaaaacctctgacacatgcagctcccggagacggtcacagcttgtctgtaagcggatgccgggagcagacaagcccgtcagggcgcgtcagcgggtgttggcgggtgtcggggctggcttaactatgcggcatcagagcagattgtactgagagtgcaccatatcgacgctctcccttatgcgactcctgcattaggaagcagcccagtagtaggttgaggccgttgagcaccgccgccgcaaggaatggtgcatgcaaggagatggcgcccaacagtcccccggccacggggcctgccaccatacccacgccgaaacaagcgctcatgagcccgaagtggcgagcccgatcttccccatcggtgatgtcggcgatataggcgccagcaaccgcacctgtggcgccggtgatgccggccacgatgcgtccggcgtagaggatctggctagcgatgaccctgctgattggttcgctgaccatttccggggtgcggaacggcgttaccagaaactcagaaggttcgtccaaccaaaccgactctgacggcagtttacgagagagatgatagggtctgcttcagtaagccagatgctacacaattaggcttgtacatattgtcgttagaacgcggctacaattaatacataaccttatgtatcatacacatacgatttaggtgacactatagaatacacctgcaggacgcgtactgagagcgctattctgaacttttcttttgttc

SEQ ID NO: 6 - DNA, 9522 bp, Artificial Sequence
  pCLD22
ccttcccttctaccacaccctaattgtaatccattttaatttcctggtcacagtcctgtctctccttccattgtaccttgcccttttctaaagagcgactgcaaagtatgtttgcgtaggtgaggatctaaaactttatgaggtacgaacatcacagaattactttgtaatttcagtttattgtaggcttggctttttggggagggtttacgtcttagacctcttagtgcttctttgtttcatggtgttctaacttcgaagcatctctgtagctttaatggattccttttctgaaagctttgctctctttcttccccctcggctttctcttaggcaagagggctaactgtaaagtaaggcttactgccttgtgtttccaaatgtgtccgaagaggaagtgtcttctgtgaatcctgttatgcatgaataacaggaaatagaaagaaattcactttcattattataaaagtaatatgttcgtttaaaaaattctaatgaagagctggagatgcaacccaggggtagagcacacactcagcatgcaggaggccctgggtccaatcttggaatctcctctcagttaacctgatctctagctgattagtagtgagtgcaagcccactttcctcttctgcctcattgctcagtgataacagctgttaaactttgtcttattctaaaactacctctgtgcaaatgctagcacaataatatatatcatatgcacatgattttttttttatcttgaaaagtaagtcagtatagctacaaagttcacttggcattgtcaacatttcacaggcgtaatattcctcctctagtactgtcctcttcattctttgtgaccaagtttggagagagtgcacaaatgccagggaggtttgtgggaaggtttctcatgttctggtaaggcgagtaagaaaatagtctcatgcaggtgaaatgagtgctatgcagtatatattataccagagaacagcaaatgaccaaattcacactgaactagttcagtaaaattggctttgtcaaagctttccttgcttaaaatgtaattccctgtcatcctagttctggtctggattcttttcctggagtcttgacttccagattccctgtggacttttgtttgagtttcaagcttttgaaatatagaaacctatctaacttaacaaacttgggagagaaaagactccagaacaactgaaaacagaccaggctaaatgaatagactttattcctctcttcttacctgcagttttcagatatgcagagttggagcggatcttagaggttgattcattcatgcctgaagaaaacacattttatagaccctgtgcccaagttcgtggtggacatcaccctttatttactaattgcactacataacaggcattttagaagactgctccagtcagagaccccgccttagaggaatctgtaaaccctgaactcctatcactcatgagcactagttatgtttggaatgccgtattaaaacaaaagttacatttctaaacttaaaattttctagcacagagacagtgggagtagctaactttgatagacatttttctactaaaagtctttctaagtacataatcttctgtaagttggaaaacagcaaaatagaacgtctcctacgtagttaatctttttgcataatttgcacatgtaggagttattagtatacgggtaagttttcactttttcccccaactggagtgtcttgtggctgggtttgaaaaagggaacgggaggccgctggaggggattggtaaatgagataaaacaccactcattcaactcagtgactcagcatttaaattttccataaaaggattaaaggaaaattaaacaaattcttaaagccaagactctggagaaacttgttggtgtgctttagttttcactgttatgactcatgaatttatgcataaattagtacatttataaaaacatagcctttttagagttttctgtttggctaaagtgccattgttagcatttggaattacctttttatgtcttatattttttccaaataaaaataaatgtttctgctgtcttactactgaaactacgttgtgagcactttaaatttctcaaagcagtttcgcctgttatacttggcgcttagtcatcgtcgtacacaacaggacctgattaagaaggctgtgctgcctctaagccgggctagattgtagccactagcaaccaggctgcaataatttccctttgatgacatcatccactgtggaagaacccagttgcttcagccagtcgaactatacagttccaacctcatcaaatatggcatctcccttgcctgctatagcagggggaggaaaaaatgccaccatctttttaatctagcaagcttctcttttcttcatctttttttttttcttttaaaaaaattctgatcatggatgcttcttccgatccctatttgccttatgacgggggaggagacaatatccccttgagggaattacataaaagaggtaagagcatccccttgctctgaatcctctgttggttgttgtgcatgcggctgggcggttctggggacaggctgtctgttgtcctcttgctgcaatgtgctgcttagttgccctgccttgttgctgtgggagaatgcgaccttcccagcagggctggccctccctgattgtttgctctgtgcagattagccctgcttcagatcacatagggctgcagactccatcttctgtgtgaaaatgctttcggtttgattgcagaaataagctgcctttacagccagctaaagtcctggtggttggttggcacctgcaaagtagtatttttgtacctctggaaacttatattttctttacacagcaatatcaagtgccggtatgccattctgttttggctgctgccaattaccatgtagactttgcaccacagagtaatagtaaaagctcctagctgcattttataacatttaaaaatagcaggaaagaagaattatttttgatttaacatgtttttgtcatttaacgtcttaactgattgacatactatattgtctgtctcgtgggtatcttgtacaacttgataggataaagcaatttagtttttttttttttttttaaatacatccagaatgtaagtcgtcagtagttttcgaacagataagtaatggtgttaatcttttggcaggctttgccttggtctccttaaagctaattaggtgttacttaattaaactgctcttttgctcattttcttaaattatttttttaaaagatagttggcatttgctgttctagaaataaacttcaagaaacattctttagccagatgacttcatgtatgagccatgttagtttgaattatttgcttggtgttataaactttatggtttaataccaacttttattatgtttacaaggtaaataaggaaaatttcaagtacattttgtatcctgagaacaaatttaagttccatagaatttaggaattacaatgtattcaacagatacttacttgtcatactgtgcctgcaaaacaataattagactctgaacaggtgcaacaattttctgtagaattagacaagtcttcttttggcaggtgttactaagtaggccatttcccaaggaacagggaatttgccaggcttttgtggtggagagaatagaatgaataaatgctgtggggagtaaagagcttgtcagaagatgattagttctgtggcaccaaaaccaagagatcagttttcctgtgagaagtaaaggaagcattgtagaaaaatagatgtgttgaagtctaccggtggagttccgcgttacataacttacggtaaatggcccgcctggctgaccgcccaacgacccccgcccattgacgtcaataatgacgtatgttcccatagtaacgccaatagggactttccattgacgtcaatgggtggagtatttacggtaaactgcccacttggcagtacatcaagtgtatcatatgccaagtacgccccctattgacgtcaatgacggtaaatggcccgcctggcattatgcccagtacatgaccttatgggactttcctacttggcagtacatctacgtattagtcatcgctattaccattgtgatgcggttttggcagtacatcaatgggcgtggatagcggtttgactcacggggatttccaagtctccaccccattgacgtcaatgggagtttgttttggcaccaaaatcaacgggactttccaaaatgtcgtaacaactccgccccattgacgcaaatgggcggtaggcgtgtacggtgggaggtctatataagcagagctcgtttagtgaaccgtcagatctacctcttccgcatcgctgtctgcgagggccagctgttggggtgagtactccctctcaaaagcgggcatgacttctgcgctaagattgtcagtttccaaaaacgaggaggatttgatattcacctggcccgcggtgatgcctttgagggtggccgcgtccatctggtcagaaaagacaatctttttgttgtcaagcttccttgatgatgtcatacttatcctgtcccttttttttccacagctcgcggttgaggacaaactcttcgcggtctttccagtactcttggatcggaaacccgtcggcctccgaacggtactccgccaccgagggacctgagcgagtccgcatcgaccggatcggaaaacctcggatccgaattcatagataactgatccagtgcccctaacgttactggccgaagccgcttggaataaggccggtgtgcgtttgtctatatgttattttccaccatattgccgtcttttggcaatgtgagggcccggaaacctggccctgtcttcttgacgagcattcctaggggtctttcccctctcgccaaaggaatgcaaggtctgttgaatgtcgtgaaggaagcagttcctctggaagcttcttgaagacaaacaacgtctgtagcgaccctttgcaggcagcggaaccccccacctggcgacaggtgcctctgcggccaaaagccacgtgtataagatacacctgcaaaggcggcacaaccccagtgccacgttgtgagttggatagttgtggaaagagtcaaatggctctcctcaagcgtattcaacaaggggctgaaggatgcccagaaggtaccccattgtatgggatctgatctggggcctcggtgcacatgctttacatgtgtttagtcgaggttaaaaaacgtctaggccccccgaaccacggggacgtggttttcctttgaaaaacacgatggccacctcagcaagttcccacttgaacaaaaacatcaagcaaatgtacttgtgcctgccccagggtgagaaagtccaagccatgtatatctgggttgatggtactggagaaggactgcgctgcaaaacccgcaccctggactgtgagcccaagtgtgtagaagagttacctgagtggaattttgatggctctagtacctttcagtctgagggctccaacagtgacatgtatctcagccctgttgccatgtttcgggaccccttccgcagagatcccaacaagctggtgttctgtgaagttttcaagtacaaccggaagcctgcagagaccaatttaaggcactcgtgtaaacggataatggacatggtgagcaaccagcacccctggtttggaatggaacaggagtatactctgatgggaacagatgggcacccttttggttggccttccaatggctttcctgggccccaaggtccgtattactgtggtgtgggcgcagacaaagcctatggcagggatatcgtggaggctcactaccgcgcctgcttgtatgctggggtcaagattacaggaacaaatgctgaggtcatgcctgcccagtgggagttccaaataggaccctgtgaaggaatccgcatgggagatcatctctgggtggcccgtttcatcttgcatcgagtatgtgaagactttggggtaatagcaacctttgaccccaagcccattcctgggaactggaatggtgcaggctgccataccaactttagcaccaaggccatgcgggaggagaatggtctgaagcacatcgaggaggccatcgagaaactaagcaagcggcaccggtaccacattcgagcctacgatcccaaggggggcctggacaatgcccgtcgtctgactgggttccacgaaacgtccaacatcaacgacttttctgctggtgtcgccaatcgcagtgccagcatccgcattccccggactgtcggccaggagaagaaaggttactttgaagaccgccgcccctctgccaattgtgacccctttgcagtgacagaagccatcgtccgcacatgccttctcaatgagactggcgacgagcccttccaatacaaaaactaatctagatccccctcgctttcttgctgtccaatttctattaaaggttcctttgttccctaagtccaactactaaactgggggatattatgaagggccttgagcatctggattctgcctaataaaaaacatttattttcattgcaatgatgtatttaaattatttctgaatattttactaaaaagggaatgtgggaggtcagtgcatttaaaacataaagaaatgaagagggggatcttcgcgacctgcaggtctccctatagtgagtcgtattaatttcgataagccagctgcattaatgaatcggccaacgcgcggggagaggcggtttgcgtattgggcgctcttccgcttcctcgctcactgactcgctgcgctcggtcgttcggctgcggcgagcggtatcagctcactcaaaggcggtaatacggttatccacagaatcaggggataacgcaggaaagaacatgtgagcaaaaggccagcaaaaggccaggaaccgtaaaaaggccgcgttgctggcgtttttccataggctccgcccccctgacgagcatcacaaaaatcgacgctcaagtcagaggtggcgaaacccgacaggactataaagataccaggcgtttccccctggaagctccctcgtgcgctctcctgttccgaccctgccgcttaccggatacctgtccgcctttctcccttcgggaagcgtggcgctttctcatagctcacgctgtaggtatctcagttcggtgtaggtcgttcgctccaagctgggctgtgtgcacgaaccccccgttcagcccgaccgctgcgccttatccggtaactatcgtcttgagtccaacccggtaagacacgacttatcgccactggcagcagccactggtaacaggattagcagagcgaggtatgtaggcggtgctacagagttcttgaagtggtggcctaactacggctacactagaaggacagtatttggtatctgcgctctgctgaagccagttaccttcggaaaaagagttggtagctcttgatccggcaaacaaaccaccgctggtagcggtggtttttttgtttgcaagcagcagattacgcgcagaaaaaaaggatctcaagaagatcctttgatcttttctacggggtctgacgctcagtggaacgaaaactcacgttaagggattttggtcatgagattatcaaaaaggatcttcacctagatccttttaaattaaaaatgaagttttaaatcaatctaaagtatatatgagtaaacttggtctgacagttaccaatgcttaatcagtgaggcacctatctcagcgatctgtctatttcgttcatccatagttgcctgactccccgtcgtgtagataactacgatacgggagggcttaccatctggccccagtgctgcaatgataccgcgagacccacgctcaccggctccagatttatcagcaataaaccagccagccggaagggccgagcgcagaagtggtcctgcaactttatccgcctccatccagtctattaattgttgccgggaagctagagtaagtagttcgccagttaatagtttgcgcaacgttgttgccattgctacaggcatcgtggtgtcacgctcgtcgtttggtatggcttcattcagctccggttcccaacgatcaaggcgagttacatgatcccccatgttgtgcaaaaaagcggttagctccttcggtcctccgatcgttgtcagaagtaagttggccgcagtgttatcactcatggttatggcagcactgcataattctcttactgtcatgccatccgtaagatgcttttctgtgactggtgagtactcaaccaagtcattctgagaatagtgtatgcggcgaccgagttgctcttgcccggcgtcaatacgggataataccgcgccacatagcagaactttaaaagtgctcatcattggaaaacgttcttcggggcgaaaactctcaaggatcttaccgctgttgagatccagttcgatgtaacccactcgtgcacccaactgatcttcagcatcttttactttcaccagcgtttctgggtgagcaaaaacaggaaggcaaaatgccgcaaaaaagggaataagggcgacacggaaatgttgaatactcatactcttcctttttcaatattattgaagcatttatcagggttattgtctcatgagcggatacatatttgaatgtatttagaaaaataaacaaataggggttccgcgcacatttccccgaaaagtgccacctgacgtctaagaaaccattattatcatgacattaacctataaaaataggcgtatcacgaggccctttcgtctcgcgcgtttcggtgatgacggtgaaaacctctgacacatgcagctcccggagacggtcacagcttgtctgtaagcggatgccgggagcagacaagcccgtcagggcgcgtcagcgggtgttggcgggtgtcggggctggcttaactatgcggcatcagagcagattgtactgagagtgcaccatatcgacgctctcccttatgcgactcctgcattaggaagcagcccagtagtaggttgaggccgttgagcaccgccgccgcaaggaatggtgcatgcaaggagatggcgcccaacagtcccccggccacggggcctgccaccatacccacgccgaaacaagcgctcatgagcccgaagtggcgagcccgatcttccccatcggtgatgtcggcgatataggcgccagcaaccgcacctgtggcgccggtgatgccggccacgatgcgtccggcgtagaggatctggctagcgatgaccctgctgattggttcgctgaccatttccggggtgcggaacggcgttaccagaaactcagaaggttcgtccaaccaaaccgactctgacggcagtttacgagagagatgatagggtctgcttcagtaagccagatgctacacaattaggcttgtacatattgtcgttagaacgcggctacaattaatacataaccttatgtatcatacacatacgatttaggtgacactatagaatacacctgcaggacgcgtactgagagcgctattctgaacttttcttttgttc

SEQ ID NO: 7 - DNA, 10767 bp, Artificial Sequence
  pCLD12
ccctagaaagataatcatattgtgacgtacgttaaagataatcatgcgtaaaattgacgcatgtgttttatcggtctgtatatcgaggtttatttattaatttgaatagatattaagttttattatatttacacttacatactaataataaattcaacaaacaatttatttatgtttatttatttattaaaaaaaaacaaaaactcaaaatttcttctataaagtaacaaaacttttatcgaatttgcagcccgggactagctagagggacagcccccccccaaagcccccagggatgtaattacgtccctcccccgctagggggcagcagcgagccgcccggggctccgctccggtccggcgctccccccgcatccccgagccggcagcgtgcggggacagcccgggcacggggaaggtggcacgggatcgctttcctctgaacgcttctcgctgctctttgagcctgcagacacctggggggatacggggaaaacttaagatccgaccggacgcgtactgagagcgctattctgaacttttcttttgttcccttcccttctaccacaccctaattgtaatccattttaatttcctggtcacagtcctgtctctccttccattgtaccttgcccttttctaaagagcgactgcaaagtatgtttgcgtaggtgaggatctaaaactttatgaggtacgaacatcacagaattactttgtaatttcagtttattgtaggcttggctttttggggagggtttacgtcttagacctcttagtgcttctttgtttcatggtgttctaacttcgaagcatctctgtagctttaatggattccttttctgaaagctttgctctctttcttccccctcggctttctcttaggcaagagggctaactgtaaagtaaggcttactgccttgtgtttccaaatgtgtccgaagaggaagtgtcttctgtgaatcctgttatgcatgaataacaggaaatagaaagaaattcactttcattattataaaagtaatatgttcgtttaaaaaattctaatgaagagctggagatgcaacccaggggtagagcacacactcagcatgcaggaggccctgggtccaatcttggaatctcctctcagttaacctgatctctagctgattagtagtgagtgcaagcccactttcctcttctgcctcattgctcagtgataacagctgttaaactttgtcttattctaaaactacctctgtgcaaatgctagcacaataatatatatcatatgcacatgattttttttttatcttgaaaagtaagtcagtatagctacaaagttcacttggcattgtcaacatttcacaggcgtaatattcctcctctagtactgtcctcttcattctttgtgaccaagtttggagagagtgcacaaatgccagggaggtttgtgggaaggtttctcatgttctggtaaggcgagtaagaaaatagtctcatgcaggtgaaatgagtgctatgcagtatatattataccagagaacagcaaatgaccaaattcacactgaactagttcagtaaaattggctttgtcaaagctttccttgcttaaaatgtaattccctgtcatcctagttctggtctggattcttttcctggagtcttgacttccagattccctgtggacttttgtttgagtttcaagcttttgaaatatagaaacctatctaacttaacaaacttgggagagaaaagactccagaacaactgaaaacagaccaggctaaatgaatagactttattcctctcttcttacctgcagttttcagatatgcagagttggagcggatcttagaggttgattcattcatgcctgaagaaaacacattttatagaccctgtgcccaagttcgtggtggacatcaccctttatttactaattgcactacataacaggcattttagaagactgctccagtcagagaccccgccttagaggaatctgtaaaccctgaactcctatcactcatgagcactagttatgtttggaatgccgtattaaaacaaaagttacatttctaaacttaaaattttctagcacagagacagtgggagtagctaactttgatagacatttttctactaaaagtctttctaagtacataatcttctgtaagttggaaaacagcaaaatagaacgtctcctacgtagttaatctttttgcataatttgcacatgtaggagttattagtatacgggtaagttttcactttttcccccaactggagtgtcttgtggctgggtttgaaaaagggaacgggaggccgctggaggggattggtaaatgagataaaacaccactcattcaactcagtgactcagcatttaaattttccataaaaggattaaaggaaaattaaacaaattcttaaagccaagactctggagaaacttgttggtgtgctttagttttcactgttatgactcatgaatttatgcataaattagtacatttataaaaacatagcctttttagagttttctgtttggctaaagtgccattgttagcatttggaattacctttttatgtcttatattttttccaaataaaaataaatgtttctgctgtcttactactgaaactacgttgtgagcactttaaatttctcaaagcagtttcgcctgttatacttggcgcttagtcatcgtcgtacacaacaggacctgattaagaaggctgtgctgcctctaagccgggctagattgtagccactagcaaccaggctgcaataatttccctttgatgacatcatccactgtggaagaacccagttgcttcagccagtcgaactatacagttccaacctcatcaaatatggcatctcccttgcctgctatagcagggggaggaaaaaatgccaccatctttttaatctagcaagcttctcttttcttcatctttttttttttcttttaaaaaaattctgatcatggatgcttcttccgatccctatttgccttatgacgggggaggagacaatatccccttgagggaattacataaaagaggtaagagcatccccttgctctgaatcctctgttggttgttgtgcatgcggctgggcggttctggggacaggctgtctgttgtcctcttgctgcaatgtgctgcttagttgccctgccttgttgctgtgggagaatgcgaccttcccagcagggctggccctccctgattgtttgctctgtgcagattagccctgcttcagatcacatagggctgcagactccatcttctgtgtgaaaatgctttcggtttgattgcagaaataagctgcctttacagccagctaaagtcctggtggttggttggcacctgcaaagtagtatttttgtacctctggaaacttatattttctttacacagcaatatcaagtgccggtatgccattctgttttggctgctgccaattaccatgtagactttgcaccacagagtaatagtaaaagctcctagctgcattttataacatttaaaaatagcaggaaagaagaattatttttgatttaacatgtttttgtcatttaacgtcttaactgattgacatactatattgtctgtctcgtgggtatcttgtacaacttgataggataaagcaatttagtttttttttttttttttaaatacatccagaatgtaagtcgtcagtagttttcgaacagataagtaatggtgttaatcttttggcaggctttgccttggtctccttaaagctaattaggtgttacttaattaaactgctcttttgctcattttcttaaattatttttttaaaagatagttggcatttgctgttctagaaataaacttcaagaaacattctttagccagatgacttcatgtatgagccatgttagtttgaattatttgcttggtgttataaactttatggtttaataccaacttttattatgtttacaaggtaaataaggaaaatttcaagtacattttgtatcctgagaacaaatttaagttccatagaatttaggaattacaatgtattcaacagatacttacttgtcatactgtgcctgcaaaacaataattagactctgaacaggtgcaacaattttctgtagaattagacaagtcttcttttggcaggtgttactaagtaggccatttcccaaggaacagggaatttgccaggcttttgtggtggagagaatagaatgaataaatgctgtggggagtaaagagcttgtcagaagatgattagttctgtggcaccaaaaccaagagatcagttttcctgtgagaagtaaaggaagcattgtagaaaaatagatgtgttgaagtctaccggtggagttccgcgttacataacttacggtaaatggcccgcctggctgaccgcccaacgacccccgcccattgacgtcaataatgacgtatgttcccatagtaacgccaatagggactttccattgacgtcaatgggtggagtatttacggtaaactgcccacttggcagtacatcaagtgtatcatatgccaagtacgccccctattgacgtcaatgacggtaaatggcccgcctggcattatgcccagtacatgaccttatgggactttcctacttggcagtacatctacgtattagtcatcgctattaccattgtgatgcggttttggcagtacatcaatgggcgtggatagcggtttgactcacggggatttccaagtctccaccccattgacgtcaatgggagtttgttttggcaccaaaatcaacgggactttccaaaatgtcgtaacaactccgccccattgacgcaaatgggcggtaggcgtgtacggtgggaggtctatataagcagagctcgtttagtgaaccgtcagatctacctcttccgcatcgctgtctgcgagggccagctgttggggtgagtactccctctcaaaagcgggcatgacttctgcgctaagattgtcagtttccaaaaacgaggaggatttgatattcacctggcccgcggtgatgcctttgagggtggccgcgtccatctggtcagaaaagacaatctttttgttgtcaagcttccttgatgatgtcatacttatcctgtcccttttttttccacagctcgcggttgaggacaaactcttcgcggtctttccagtactcttggatcggaaacccgtcggcctccgaacggtactccgccaccgagggacctgagcgagtccgcatcgaccggatcggaaaacctcggatccgaattcatagataactgatccagtgcccctaacgttactggccgaagccgcttggaataaggccggtgtgcgtttgtctatatgttattttccaccatattgccgtcttttggcaatgtgagggcccggaaacctggccctgtcttcttgacgagcattcctaggggtctttcccctctcgccaaaggaatgcaaggtctgttgaatgtcgtgaaggaagcagttcctctggaagcttcttgaagacaaacaacgtctgtagcgaccctttgcaggcagcggaaccccccacctggcgacaggtgcctctgcggccaaaagccacgtgtataagatacacctgcaaaggcggcacaaccccagtgccacgttgtgagttggatagttgtggaaagagtcaaatggctctcctcaagcgtattcaacaaggggctgaaggatgcccagaaggtaccccattgtatgggatctgatctggggcctcggtgcacatgctttacatgtgtttagtcgaggttaaaaaacgtctaggccccccgaaccacggggacgtggttttcctttgaaaaacacgatgataatatggccacaaccatggccacctcagcaagttcccacttgaacaaaaacatcaagcaaatgtacttgtgcctgccccagggtgagaaagtccaagccatgtatatctgggttgatggtactggagaaggactgcgctgcaaaacccgcaccctggactgtgagcccaagtgtgtagaagagttacctgagtggaattttgatggctctagtacctttcagtctgagggctccaacagtgacatgtatctcagccctgttgccatgtttcgggaccccttccgcagagatcccaacaagctggtgttctgtgaagttttcaagtacaaccggaagcctgcagagaccaatttaaggcactcgtgtaaacggataatggacatggtgagcaaccagcacccctggtttggaatggaacaggagtatactctgatgggaacagatgggcacccttttggttggccttccaatggctttcctgggccccaaggtccgtattactgtggtgtgggcgcagacaaagcctatggcagggatatcgtggaggctcactaccgcgcctgcttgtatgctggggtcaagattacaggaacaaatgctgaggtcatgcctgcccagtgggagttccaaataggaccctgtgaaggaatccgcatgggagatcatctctgggtggcccgtttcatcttgcatcgagtatgtgaagactttggggtaatagcaacctttgaccccaagcccattcctgggaactggaatggtgcaggctgccataccaactttagcaccaaggccatgcgggaggagaatggtctgaagcacatcgaggaggccatcgagaaactaagcaagcggcaccggtaccacattcgagcctacgatcccaaggggggcctggacaatgcccgtcgtctgactgggttccacgaaacgtccaacatcaacgacttttctgctggtgtcgccaatcgcagtgccagcatccgcattccccggactgtcggccaggagaagaaaggttactttgaagaccgccgcccctctgccaattgtgacccctttgcagtgacagaagccatcgtccgcacatgccttctcaatgagactggcgacgagcccttccaatacaaaaactaatctagatccccctcgctttcttgctgtccaatttctattaaaggttcctttgttccctaagtccaactactaaactgggggatattatgaagggccttgagcatctggattctgcctaataaaaaacatttattttcattgcaatgatgtatttaaattatttctgaatattttactaaaaagggaatgtgggaggtcagtgcatttaaaacataaagaaatgaagagggggatcttcgcgatactgcatcgatgagggacagcccccccccaaagcccccagggatgtaattacgtccctcccccgctagggggcagcagcgagccgcccggggctccgctccggtccggcgctccccccgcatccccgagccggcagcgtgcggggacagcccgggcacggggaaggtggcacgggatcgctttcctctgaacgcttctcgctgctctttgagcctgcagacacctggggggatacggggaaaatagacaccgcggtggagctccagcttttgttccctttagtgagggttaattagttcttaatacgactcactatagggcgaattggctaccgggccgcccatcgagggtatcataagcttatatctataacaagaaaatatatatataataagttatcacgtaagtagaacatgaaataacaatataattatcgtatgagttaaatcttaaaagtcacgtaaaagataatcatgcgtcattttgactcacgcggtcgttatagttcaaaatcagtgacacttaccgcattgacaagcacgcctcacgggagctccaagcggcgactgagatgtcctaaatgcacagcgacggattcgcgctatttagaaagagagagcaatatttcaagaatgcatgcgtcaattttacgcagactatctttctagggttaaatcgatagatgcgatcctgcaggtctccctatagtgagtcgtattaatttcgataagccagctgcattaatgaatcggccaacgcgcggggagaggcggtttgcgtattgggcgctcttccgcttcctcgctcactgactcgctgcgctcggtcgttcggctgcggcgagcggtatcagctcactcaaaggcggtaatacggttatccacagaatcaggggataacgcaggaaagaacatgtgagcaaaaggccagcaaaaggccaggaaccgtaaaaaggccgcgttgctggcgtttttccataggctccgcccccctgacgagcatcacaaaaatcgacgctcaagtcagaggtggcgaaacccgacaggactataaagataccaggcgtttccccctggaagctccctcgtgcgctctcctgttccgaccctgccgcttaccggatacctgtccgcctttctcccttcgggaagcgtggcgctttctcatagctcacgctgtaggtatctcagttcggtgtaggtcgttcgctccaagctgggctgtgtgcacgaaccccccgttcagcccgaccgctgcgccttatccggtaactatcgtcttgagtccaacccggtaagacacgacttatcgccactggcagcagccactggtaacaggattagcagagcgaggtatgtaggcggtgctacagagttcttgaagtggtggcctaactacggctacactagaaggacagtatttggtatctgcgctctgctgaagccagttaccttcggaaaaagagttggtagctcttgatccggcaaacaaaccaccgctggtagcggtggtttttttgtttgcaagcagcagattacgcgcagaaaaaaaggatctcaagaagatcctttgatcttttctacggggtctgacgctcagtggaacgaaaactcacgttaagggattttggtcatgagattatcaaaaaggatcttcacctagatccttttaaattaaaaatgaagttttaaatcaatctaaagtatatatgagtaaacttggtctgacagttaccaatgcttaatcagtgaggcacctatctcagcgatctgtctatttcgttcatccatagttgcctgactccccgtcgtgtagataactacgatacgggagggcttaccatctggccccagtgctgcaatgataccgcgagacccacgctcaccggctccagatttatcagcaataaaccagccagccggaagggccgagcgcagaagtggtcctgcaactttatccgcctccatccagtctattaattgttgccgggaagctagagtaagtagttcgccagttaatagtttgcgcaacgttgttgccattgctacaggcatcgtggtgtcacgctcgtcgtttggtatggcttcattcagctccggttcccaacgatcaaggcgagttacatgatcccccatgttgtgcaaaaaagcggttagctccttcggtcctccgatcgttgtcagaagtaagttggccgcagtgttatcactcatggttatggcagcactgcataattctcttactgtcatgccatccgtaagatgcttttctgtgactggtgagtactcaaccaagtcattctgagaatagtgtatgcggcgaccgagttgctcttgcccggcgtcaatacgggataataccgcgccacatagcagaactttaaaagtgctcatcattggaaaacgttcttcggggcgaaaactctcaaggatcttaccgctgttgagatccagttcgatgtaacccactcgtgcacccaactgatcttcagcatcttttactttcaccagcgtttctgggtgagcaaaaacaggaaggcaaaatgccgcaaaaaagggaataagggcgacacggaaatgttgaatactcatactcttcctttttcaatattattgaagcatttatcagggttattgtctcatgagcggatacatatttgaatgtatttagaaaaataaacaaataggggttccgcgcacatttccccgaaaagtgccacctgacgtctaagaaaccattattatcatgacattaacctataaaaataggcgtatcacgaggccctttcgtctcgcgcgtttcggtgatgacggtgaaaacctctgacacatgcagctcccggagacggtcacagcttgtctgtaagcggatgccgggagcagacaagcccgtcagggcgcgtcagcgggtgttggcgggtgtcggggctggcttaactatgcggcatcagagcagattgtactgagagtgcaccatatcgacgctctcccttatgcgactcctgcattaggaagcagcccagtagtaggttgaggccgttgagcaccgccgccgcaaggaatggtgcatgcaaggagatggcgcccaacagtcccccggccacggggcctgccaccatacccacgccgaaacaagcgctcatgagcccgaagtggcgagcccgatcttccccatcggtgatgtcggcgatataggcgccagcaaccgcacctgtggcgccggtgatgccggccacgatgcgtccggcgtagaggatctggctagcgatgaccctgctgattggttcgctgaccatttccggggtgcggaacggcgttaccagaaactcagaaggttcgtccaaccaaaccgactctgacggcagtttacgagagagatgatagggtctgcttcagtaagccagatgctacacaattaggcttgtacatattgtcgttagaacgcggctacaattaatacataaccttatgtatcatacacatacgatttaggtgacactatagaatacacctgcaggacgtcccaatgatcttaagttaa

SEQ ID NO: 8 - DNA, 10747 bp, Artificial Sequence
  pCLD14
ccctagaaagataatcatattgtgacgtacgttaaagataatcatgcgtaaaattgacgcatgtgttttatcggtctgtatatcgaggtttatttattaatttgaatagatattaagttttattatatttacacttacatactaataataaattcaacaaacaatttatttatgtttatttatttattaaaaaaaaacaaaaactcaaaatttcttctataaagtaacaaaacttttatcgaatttgcagcccgggactagctagagggacagcccccccccaaagcccccagggatgtaattacgtccctcccccgctagggggcagcagcgagccgcccggggctccgctccggtccggcgctccccccgcatccccgagccggcagcgtgcggggacagcccgggcacggggaaggtggcacgggatcgctttcctctgaacgcttctcgctgctctttgagcctgcagacacctggggggatacggggaaaacttaagatccgaccggacgcgtactgagagcgctattctgaacttttcttttgttcccttcccttctaccacaccctaattgtaatccattttaatttcctggtcacagtcctgtctctccttccattgtaccttgcccttttctaaagagcgactgcaaagtatgtttgcgtaggtgaggatctaaaactttatgaggtacgaacatcacagaattactttgtaatttcagtttattgtaggcttggctttttggggagggtttacgtcttagacctcttagtgcttctttgtttcatggtgttctaacttcgaagcatctctgtagctttaatggattccttttctgaaagctttgctctctttcttccccctcggctttctcttaggcaagagggctaactgtaaagtaaggcttactgccttgtgtttccaaatgtgtccgaagaggaagtgtcttctgtgaatcctgttatgcatgaataacaggaaatagaaagaaattcactttcattattataaaagtaatatgttcgtttaaaaaattctaatgaagagctggagatgcaacccaggggtagagcacacactcagcatgcaggaggccctgggtccaatcttggaatctcctctcagttaacctgatctctagctgattagtagtgagtgcaagcccactttcctcttctgcctcattgctcagtgataacagctgttaaactttgtcttattctaaaactacctctgtgcaaatgctagcacaataatatatatcatatgcacatgattttttttttatcttgaaaagtaagtcagtatagctacaaagttcacttggcattgtcaacatttcacaggcgtaatattcctcctctagtactgtcctcttcattctttgtgaccaagtttggagagagtgcacaaatgccagggaggtttgtgggaaggtttctcatgttctggtaaggcgagtaagaaaatagtctcatgcaggtgaaatgagtgctatgcagtatatattataccagagaacagcaaatgaccaaattcacactgaactagttcagtaaaattggctttgtcaaagctttccttgcttaaaatgtaattccctgtcatcctagttctggtctggattcttttcctggagtcttgacttccagattccctgtggacttttgtttgagtttcaagcttttgaaatatagaaacctatctaacttaacaaacttgggagagaaaagactccagaacaactgaaaacagaccaggctaaatgaatagactttattcctctcttcttacctgcagttttcagatatgcagagttggagcggatcttagaggttgattcattcatgcctgaagaaaacacattttatagaccctgtgcccaagttcgtggtggacatcaccctttatttactaattgcactacataacaggcattttagaagactgctccagtcagagaccccgccttagaggaatctgtaaaccctgaactcctatcactcatgagcactagttatgtttggaatgccgtattaaaacaaaagttacatttctaaacttaaaattttctagcacagagacagtgggagtagctaactttgatagacatttttctactaaaagtctttctaagtacataatcttctgtaagttggaaaacagcaaaatagaacgtctcctacgtagttaatctttttgcataatttgcacatgtaggagttattagtatacgggtaagttttcactttttcccccaactggagtgtcttgtggctgggtttgaaaaagggaacgggaggccgctggaggggattggtaaatgagataaaacaccactcattcaactcagtgactcagcatttaaattttccataaaaggattaaaggaaaattaaacaaattcttaaagccaagactctggagaaacttgttggtgtgctttagttttcactgttatgactcatgaatttatgcataaattagtacatttataaaaacatagcctttttagagttttctgtttggctaaagtgccattgttagcatttggaattacctttttatgtcttatattttttccaaataaaaataaatgtttctgctgtcttactactgaaactacgttgtgagcactttaaatttctcaaagcagtttcgcctgttatacttggcgcttagtcatcgtcgtacacaacaggacctgattaagaaggctgtgctgcctctaagccgggctagattgtagccactagcaaccaggctgcaataatttccctttgatgacatcatccactgtggaagaacccagttgcttcagccagtcgaactatacagttccaacctcatcaaatatggcatctcccttgcctgctatagcagggggaggaaaaaatgccaccatctttttaatctagcaagcttctcttttcttcatctttttttttttcttttaaaaaaattctgatcatggatgcttcttccgatccctatttgccttatgacgggggaggagacaatatccccttgagggaattacataaaagaggtaagagcatccccttgctctgaatcctctgttggttgttgtgcatgcggctgggcggttctggggacaggctgtctgttgtcctcttgctgcaatgtgctgcttagttgccctgccttgttgctgtgggagaatgcgaccttcccagcagggctggccctccctgattgtttgctctgtgcagattagccctgcttcagatcacatagggctgcagactccatcttctgtgtgaaaatgctttcggtttgattgcagaaataagctgcctttacagccagctaaagtcctggtggttggttggcacctgcaaagtagtatttttgtacctctggaaacttatattttctttacacagcaatatcaagtgccggtatgccattctgttttggctgctgccaattaccatgtagactttgcaccacagagtaatagtaaaagctcctagctgcattttataacatttaaaaatagcaggaaagaagaattatttttgatttaacatgtttttgtcatttaacgtcttaactgattgacatactatattgtctgtctcgtgggtatcttgtacaacttgataggataaagcaatttagtttttttttttttttttaaatacatccagaatgtaagtcgtcagtagttttcgaacagataagtaatggtgttaatcttttggcaggctttgccttggtctccttaaagctaattaggtgttacttaattaaactgctcttttgctcattttcttaaattatttttttaaaagatagttggcatttgctgttctagaaataaacttcaagaaacattctttagccagatgacttcatgtatgagccatgttagtttgaattatttgcttggtgttataaactttatggtttaataccaacttttattatgtttacaaggtaaataaggaaaatttcaagtacattttgtatcctgagaacaaatttaagttccatagaatttaggaattacaatgtattcaacagatacttacttgtcatactgtgcctgcaaaacaataattagactctgaacaggtgcaacaattttctgtagaattagacaagtcttcttttggcaggtgttactaagtaggccatttcccaaggaacagggaatttgccaggcttttgtggtggagagaatagaatgaataaatgctgtggggagtaaagagcttgtcagaagatgattagttctgtggcaccaaaaccaagagatcagttttcctgtgagaagtaaaggaagcattgtagaaaaatagatgtgttgaagtctaccggtggagttccgcgttacataacttacggtaaatggcccgcctggctgaccgcccaacgacccccgcccattgacgtcaataatgacgtatgttcccatagtaacgccaatagggactttccattgacgtcaatgggtggagtatttacggtaaactgcccacttggcagtacatcaagtgtatcatatgccaagtacgccccctattgacgtcaatgacggtaaatggcccgcctggcattatgcccagtacatgaccttatgggactttcctacttggcagtacatctacgtattagtcatcgctattaccattgtgatgcggttttggcagtacatcaatgggcgtggatagcggtttgactcacggggatttccaagtctccaccccattgacgtcaatgggagtttgttttggcaccaaaatcaacgggactttccaaaatgtcgtaacaactccgccccattgacgcaaatgggcggtaggcgtgtacggtgggaggtctatataagcagagctcgtttagtgaaccgtcagatctacctcttccgcatcgctgtctgcgagggccagctgttggggtgagtactccctctcaaaagcgggcatgacttctgcgctaagattgtcagtttccaaaaacgaggaggatttgatattcacctggcccgcggtgatgcctttgagggtggccgcgtccatctggtcagaaaagacaatctttttgttgtcaagcttccttgatgatgtcatacttatcctgtcccttttttttccacagctcgcggttgaggacaaactcttcgcggtctttccagtactcttggatcggaaacccgtcggcctccgaacggtactccgccaccgagggacctgagcgagtccgcatcgaccggatcggaaaacctcggatccgaattcatagataactgatccagtgcccctaacgttactggccgaagccgcttggaataaggccggtgtgcgtttgtctatatgttattttccaccatattgccgtcttttggcaatgtgagggcccggaaacctggccctgtcttcttgacgagcattcctaggggtctttcccctctcgccaaaggaatgcaaggtctgttgaatgtcgtgaaggaagcagttcctctggaagcttcttgaagacaaacaacgtctgtagcgaccctttgcaggcagcggaaccccccacctggcgacaggtgcctctgcggccaaaagccacgtgtataagatacacctgcaaaggcggcacaaccccagtgccacgttgtgagttggatagttgtggaaagagtcaaatggctctcctcaagcgtattcaacaaggggctgaaggatgcccagaaggtaccccattgtatgggatctgatctggggcctcggtgcacatgctttacatgtgtttagtcgaggttaaaaaacgtctaggccccccgaaccacggggacgtggttttcctttgaaaaacacgatggccacctcagcaagttcccacttgaacaaaaacatcaagcaaatgtacttgtgcctgccccagggtgagaaagtccaagccatgtatatctgggttgatggtactggagaaggactgcgctgcaaaacccgcaccctggactgtgagcccaagtgtgtagaagagttacctgagtggaattttgatggctctagtacctttcagtctgagggctccaacagtgacatgtatctcagccctgttgccatgtttcgggaccccttccgcagagatcccaacaagctggtgttctgtgaagttttcaagtacaaccggaagcctgcagagaccaatttaaggcactcgtgtaaacggataatggacatggtgagcaaccagcacccctggtttggaatggaacaggagtatactctgatgggaacagatgggcacccttttggttggccttccaatggctttcctgggccccaaggtccgtattactgtggtgtgggcgcagacaaagcctatggcagggatatcgtggaggctcactaccgcgcctgcttgtatgctggggtcaagattacaggaacaaatgctgaggtcatgcctgcccagtgggagttccaaataggaccctgtgaaggaatccgcatgggagatcatctctgggtggcccgtttcatcttgcatcgagtatgtgaagactttggggtaatagcaacctttgaccccaagcccattcctgggaactggaatggtgcaggctgccataccaactttagcaccaaggccatgcgggaggagaatggtctgaagcacatcgaggaggccatcgagaaactaagcaagcggcaccggtaccacattcgagcctacgatcccaaggggggcctggacaatgcccgtcgtctgactgggttccacgaaacgtccaacatcaacgacttttctgctggtgtcgccaatcgcagtgccagcatccgcattccccggactgtcggccaggagaagaaaggttactttgaagaccgccgcccctctgccaattgtgacccctttgcagtgacagaagccatcgtccgcacatgccttctcaatgagactggcgacgagcccttccaatacaaaaactaatctagatccccctcgctttcttgctgtccaatttctattaaaggttcctttgttccctaagtccaactactaaactgggggatattatgaagggccttgagcatctggattctgcctaataaaaaacatttattttcattgcaatgatgtatttaaattatttctgaatattttactaaaaagggaatgtgggaggtcagtgcatttaaaacataaagaaatgaagagggggatcttcgcgatactgcatcgatgagggacagcccccccccaaagcccccagggatgtaattacgtccctcccccgctagggggcagcagcgagccgcccggggctccgctccggtccggcgctccccccgcatccccgagccggcagcgtgcggggacagcccgggcacggggaaggtggcacgggatcgctttcctctgaacgcttctcgctgctctttgagcctgcagacacctggggggatacggggaaaatagacaccgcggtggagctccagcttttgttccctttagtgagggttaattagttcttaatacgactcactatagggcgaattggctaccgggccgcccatcgagggtatcataagcttatatctataacaagaaaatatatatataataagttatcacgtaagtagaacatgaaataacaatataattatcgtatgagttaaatcttaaaagtcacgtaaaagataatcatgcgtcattttgactcacgcggtcgttatagttcaaaatcagtgacacttaccgcattgacaagcacgcctcacgggagctccaagcggcgactgagatgtcctaaatgcacagcgacggattcgcgctatttagaaagagagagcaatatttcaagaatgcatgcgtcaattttacgcagactatctttctagggttaaatcgatagatgcgatcctgcaggtctccctatagtgagtcgtattaatttcgataagccagctgcattaatgaatcggccaacgcgcggggagaggcggtttgcgtattgggcgctcttccgcttcctcgctcactgactcgctgcgctcggtcgttcggctgcggcgagcggtatcagctcactcaaaggcggtaatacggttatccacagaatcaggggataacgcaggaaagaacatgtgagcaaaaggccagcaaaaggccaggaaccgtaaaaaggccgcgttgctggcgtttttccataggctccgcccccctgacgagcatcacaaaaatcgacgctcaagtcagaggtggcgaaacccgacaggactataaagataccaggcgtttccccctggaagctccctcgtgcgctctcctgttccgaccctgccgcttaccggatacctgtccgcctttctcccttcgggaagcgtggcgctttctcatagctcacgctgtaggtatctcagttcggtgtaggtcgttcgctccaagctgggctgtgtgcacgaaccccccgttcagcccgaccgctgcgccttatccggtaactatcgtcttgagtccaacccggtaagacacgacttatcgccactggcagcagccactggtaacaggattagcagagcgaggtatgtaggcggtgctacagagttcttgaagtggtggcctaactacggctacactagaaggacagtatttggtatctgcgctctgctgaagccagttaccttcggaaaaagagttggtagctcttgatccggcaaacaaaccaccgctggtagcggtggtttttttgtttgcaagcagcagattacgcgcagaaaaaaaggatctcaagaagatcctttgatcttttctacggggtctgacgctcagtggaacgaaaactcacgttaagggattttggtcatgagattatcaaaaaggatcttcacctagatccttttaaattaaaaatgaagttttaaatcaatctaaagtatatatgagtaaacttggtctgacagttaccaatgcttaatcagtgaggcacctatctcagcgatctgtctatttcgttcatccatagttgcctgactccccgtcgtgtagataactacgatacgggagggcttaccatctggccccagtgctgcaatgataccgcgagacccacgctcaccggctccagatttatcagcaataaaccagccagccggaagggccgagcgcagaagtggtcctgcaactttatccgcctccatccagtctattaattgttgccgggaagctagagtaagtagttcgccagttaatagtttgcgcaacgttgttgccattgctacaggcatcgtggtgtcacgctcgtcgtttggtatggcttcattcagctccggttcccaacgatcaaggcgagttacatgatcccccatgttgtgcaaaaaagcggttagctccttcggtcctccgatcgttgtcagaagtaagttggccgcagtgttatcactcatggttatggcagcactgcataattctcttactgtcatgccatccgtaagatgcttttctgtgactggtgagtactcaaccaagtcattctgagaatagtgtatgcggcgaccgagttgctcttgcccggcgtcaatacgggataataccgcgccacatagcagaactttaaaagtgctcatcattggaaaacgttcttcggggcgaaaactctcaaggatcttaccgctgttgagatccagttcgatgtaacccactcgtgcacccaactgatcttcagcatcttttactttcaccagcgtttctgggtgagcaaaaacaggaaggcaaaatgccgcaaaaaagggaataagggcgacacggaaatgttgaatactcatactcttcctttttcaatattattgaagcatttatcagggttattgtctcatgagcggatacatatttgaatgtatttagaaaaataaacaaataggggttccgcgcacatttccccgaaaagtgccacctgacgtctaagaaaccattattatcatgacattaacctataaaaataggcgtatcacgaggccctttcgtctcgcgcgtttcggtgatgacggtgaaaacctctgacacatgcagctcccggagacggtcacagcttgtctgtaagcggatgccgggagcagacaagcccgtcagggcgcgtcagcgggtgttggcgggtgtcggggctggcttaactatgcggcatcagagcagattgtactgagagtgcaccatatcgacgctctcccttatgcgactcctgcattaggaagcagcccagtagtaggttgaggccgttgagcaccgccgccgcaaggaatggtgcatgcaaggagatggcgcccaacagtcccccggccacggggcctgccaccatacccacgccgaaacaagcgctcatgagcccgaagtggcgagcccgatcttccccatcggtgatgtcggcgatataggcgccagcaaccgcacctgtggcgccggtgatgccggccacgatgcgtccggcgtagaggatctggctagcgatgaccctgctgattggttcgctgaccatttccggggtgcggaacggcgttaccagaaactcagaaggttcgtccaaccaaaccgactctgacggcagtttacgagagagatgatagggtctgcttcagtaagccagatgctacacaattaggcttgtacatattgtcgttagaacgcggctacaattaatacataaccttatgtatcatacacatacgatttaggtgacactatagaatacacctgcaggacgtcccaatgatcttaagttaa

SEQ ID NO: 9 - DNA, 63 bp, Artificial Sequence
  5'ITR
ccctagaaagataatcatattgtgacgtacgttaaagataatcatgcgtaaaattgacgcatg

SEQ ID NO: 10 - DNA, 35 bp, Artificial Sequence
  3'ITR
catgcgtcaattttacgcagactatctttctaggg

SEQ ID NO: 11 - DNA, 1211 bp, Artificial Sequence
  HS4 Insulator
gagctcacggggacagcccccccccaaagcccccagggatgtaattacgtccctcccccgctagggggcagcagcgagccgcccggggctccgctccggtccggcgctccccccgcatccccgagccggcagcgtgcggggacagcccgggcacggggaaggtggcacgggatcgctttcctctgaacgcttctcgctgctctttgagcctgcagacacctggggggatacggggaaaaagctttaggctgaaagagagatttagaatgacagaatcatagaacggcctgggttgcaaaggagcacagtgctcatccagatccaaccccctgctatgtgcagggtcatcaaccagcagcccaggctgcccagagccacatccagcctggccttgaatgcctgcagggatggggcatccacagcctccttgggcaacctgttcagtgcgtcaccaccctctgggggaaaaactgcctcctcatatccaacccaaacctcccctgtctcagtgtaaagccattcccccttgtcctatcaagggggagtttgctgtgacattgttggtctggggtgacacatgtttgccaattcagtgcatcacggagaggcagatcttggggataaggaagtgcaggacagcatggacgtgggacatgcaggtgttgagggctctgggacactctccaagtcacagcgttcagaacagccttaaggataagaagataggatagaaggacaaagagcaagttaaaacccagcatggagaggagcacaaaaaggccacagacactgctggtccctgtgtctgagcctgcatgtttgatggtgtctggatgcaagcagaaggggtggaagagcttgcctggagagatacagctgggtcagtaggactgggacaggcagctggagaattgccatgtagatgttcatacaatcgtcaaatcatgaaggctggaaaagccctccaagatccccaagaccaaccccaacccacccaccgtgcccactggccatgtccctcagtgccacatccccacagttcttcatcacctccagggacggtgacccccccacctccgtgggcagctgtgccactgcagcaccgctctttggagaaggtaaatcttgctaaatccagcccgaccctcccctggcacaacgtaaggccattatctctcatccaactccaggacggagtcagtgagaatatt

SEQ ID NO: 12 - DNA, 5837 bp, Artificial Sequence
  EASE
gaattctgaacttttcttttgttcccttcccttctaccacaccctaattgtaatccattttaatttcctggtcacagtcctgtctctccttccattgtaccttgcccttttctaaagagcgactgcaaagtatgtttgcgtaggtgaggatctaaaactttatgaggtacgaacatcacagaattactttgtaatttcagtttattgtaggcttggctttttggggagggtttacgtcttagacctcttagtgcttctttgtttcatggtgttctaacttcgaagcatctctgtagctttaatggattccttttctgaaagctttgctctctttcttccccctcggctttctcttaggcaagagggctaactgtaaagtaaggcttactgccttgtgtttccaaatgtgtccgaagaggaagtgtcttctgtgaatcctgttatgcatgaataacaggaaatagaaagaaattcactttcattattataaaagtaatatgttcgtttaaaaaattctaatgaagagctggagatgcaacccaggggtagagcacacactcagcatgcaggaggccctgggtccaatcttggaatctcctctcagttaacctgatctctagctgattagtagtgagtgcaagcccactttcctcttctgcctcattgctcagtgataacagctgttaaactttgtcttattctaaaactacctctgtgcaaatgctagcacaataatatatatcatatgcacatgattttttttttatcttgaaaagtaagtcagtatagctacaaagttcacttggcattgtcaacatttcacaggcgtaatattcctcctctagtactgtcctcttcattctttgtgaccaagtttggagagagtgcacaaatgccagggaggtttgtgggaaggtttctcatgttctggtaaggcgagtaagaaaatagtctcatgcaggtgaaatgagtgctatgcagtatatattataccagagaacagcaaatgaccaaattcacactgaactagttcagtaaaattggctttgtcaaagctttccttgcttaaaatgtaattccctgtcatcctagttctggtctggattcttttcctggagtcttgacttccagattccctgtggacttttgtttgagtttcaagcttttgaaatatagaaacctatctaacttaacaaacttgggagagaaaagactccagaacaactgaaaacagaccaggctaaatgaatagactttattcctctcttcttacctgcagttttcagatatgcagagttggagcggatcttagaggttgattcattcatgcctgaagaaaacacattttatagaccctgtgcccaagttcgtggtggacatcaccctttatttactaattgcactacataacaggcattttagaagactgctccagtcagagaccccgccttagaggaatctgtaaaccctgaactcctatcactcatgagcactagttatgtttggaatgccgtattaaaacaaaagttacatttctaaacttaaaattttctagcacagagacagtgggagtagctaactttgatagacatttttctactaaaagtctttctaagtacataatcttctgtaagttggaaaacagcaaaatagaacgtctcctacgtagttaatctttttgcataatttgcacatgtaggagttattagtatacgggtaagttttcactttttcccccaactggagtgtcttgtggctgggtttgaaaaagggaacgggaggccgctggaggggattggtaaatgagataaaacaccactcattcaactcagtgactcagcatttaaattttccataaaaggattaaaggaaaattaaacaaattcttaaagccaagactctggagaaacttgttggtgtgctttagttttcactgttatgactcatgaatttatgcataaattagtacatttataaaaacatagcctttttagagttttctgtttggctaaagtgccattgttagcatttggaattacctttttatgtcttatattttttccaaataaaaataaatgtttctgctgtcttactactgaaactacgttgtgagcactttaaatttctcaaagcagtttcgcctgttatacttggcgcttagtcatcgtcgtacacaacaggacctgattaagaaggctgtgctgcctctaagccgggctagattgtagccactagcaaccaggctgcaataatttccctttgatgacatcatccactgtggaagaacccagttgcttcagccagtcgaactatacagttccaacctcatcaaatatggcatctcccttgcctgctatagcagggggaggaaaaaatgccaccatctttttaatctagcaagcttctcttttcttcatctttttttttttcttttaaaaaaattctgatcatggatgcttcttccgatccctatttgccttatgacgggggaggagacaatatccccttgagggaattacataaaagaggtaagagcatccccttgctctgaatcctctgttggttgttgtgcatgcggctgggcggttctggggacaggctgtctgttgtcctcttgctgcaatgtgctgcttagttgccctgccttgttgctgtgggagaatgcgaccttcccagcagggctggccctccctgattgtttgctctgtgcagattagccctgcttcagatcacatagggctgcagactccatcttctgtgtgaaaatgctttcggtttgattgcagaaataagctgcctttacagccagctaaagtcctggtggttggttggcacctgcaaagtagtatttttgtacctctggaaacttatattttctttacacagcaatatcaagtgccggtatgccattctgttttggctgctgccaattaccatgtagactttgcaccacagagtaatagtaaaagctcctagctgcattttataacatttaaaaatagcaggaaagaagaattatttttgatttaacatgtttttgtcatttaacgtcttaactgattgacatactatattgtctgtctcgtgggtatcttgtacaacttgataggataaagcaatttagtttttttttttttttttaaatacatccagaatgtaagtcgtcagtagttttcgaacagataagtaatggtgttaatcttttggcaggctttgccttggtctccttaaagctaattaggtgttacttaattaaactgctcttttgctcattttcttaaattatttttttaaaagatagttggcatttgctgttctagaaataaacttcaagaaacattctttagccagatgacttcatgtatgagccatgttagtttgaattatttgcttggtgttataaactttatggtttaataccaacttttattatgtttacaaggtaaataaggaaaatttcaagtacattttgtatcctgagaacaaatttaagttccatagaatttaggaattacaatgtattcaacagatacttacttgtcatactgtgcctgcaaaacaataattagactctgaacaggtgcaacaattttctgtagaattctgtgcttagtaaaaggttgctttttatattttgagagaaatctatttaaagatcatggcccatattttgtgcatatttttttctgtataccatttccatatatgtgtgtgtgtgtacatatatgtatatatataaaatgttagaacatttgaggaaatagctaaaagtacaaaagtaatgttttctaattttttactccccgaggttatttcttttttccttgttttcctttctctttgttcctatcatcagtttctagtaatactcttattgaacagtgattattcaaatgtcacattatttattaatcagcatttaaatggtaaaaccagacagaccatactttctctgagtgatgacaacatccatttttagtaatgataaactagaagggtcaggcttgatagtctttgtcaggactaatttatagactgtaaaggccaaaagaaataagaaatgtcaaaactcttgtgaaactagacatacagatattaccaagagagaaactagaaaaaaaaattctgtgacatggccttaatttgccaggcaccatcgtgaaggcctaaacccctcttagaagctcactcagatgccatcctgcttctctgatgagacttcctgtcaatacaaacatggtttaggaagaatgagtgtttgcagtataaaccagttatttactagccttactttaagaatatactgtagtgtccttgagagagaaggtgtttgttttctgtaatttatgacccttttgaaaccatagatcagcacaaaggaactggggatatggaaatgggaacataacttaaatccagaaaagtgaatcagattccctgtgaggacaaaatgcaatatttagaaataggatctttaggctgggagggagaaaagaggaaaaaaatgaaagtataacatttttcataagtataagatttcataaaaaaatgaaatctataacatagagggtgttgataaagtaagcatggatatgtttagtaaagccgacagagctaagaattagctttgtgagtaattggacttaatcaaacttttcaaggtgggatacaaatgaataattgtagaataaatggataaaagaatatgaataaaatgaatagtgagtaaaaattaaaaatgaagctttttacttaagtgcatattgtagtggctagaacaaatagattcaaaatagaaatcatttatatattcttgattagaagataaaatgttattttagaaatagccatctttggaagtaaatttgctatgttgaacaaccaggttttcataatttgtctcttattttttttcaggaagaaaaaaaaacttgacttatttgtactgctaagttttattcaatgtgcttgcttgcttaaatttttaatgaagttttagtcatttggtggtcaaattccttttatctactaatcgcttttcgtggctttggcttttaaaattgtatttactgcatttatttgtgtgtattaggagtcaggtggccatatgtgccatggcatgtgtatggaagcacttgtggacatgaatcttctctttccacatgtgtgggccactggaatcaaactagtgtcaggcttggcagcaatttttaatgcactgagccttctcaccaccccctggacttttgtggggcagaaggggacaagtttaatattttatttactccatgtagaaagcctttaaaaaatgtagaaagcctttaaactacctattgttttatttgaattatgaagctcttgtgtttatataaattacagttaggtactgtggagactaatggtagctacaatagtaatattaatagctaaaacttagtagaatctgattgagttaatttggccctttccatcataaggtactcttcccaagcatcacatgacctgtgcttaagtctggtgggggcttatggctttgatattgaaaacaaatcgtcaaggatgttaatttcttgttactgctattacactgaattttctatggctctttaggagaggaagagacaagtcttcttttggcaggtgttactaagtaggccatttcccaaggaacagggaatttgccaggcttttgtggtggagagaatagaatgaataaatgctgtggggagtaaagagcttgtcagaagatgattagttctgtggcaccaaaaccaagagatcagttttcctgtgagaagtaaaggaagcattgtagaaaaatagatgtgttgaagtct

SEQ ID NO: 13 - DNA, 280 bp, Artificial Sequence
  Beta-globin polyA
tgccctggcccacaagtatcactaagctcgctttcttgctgtccaatttctattaaaggttcctttgttccctaagtccaactactaaactgggggatattatgaagggccttgagcatctggattctgcctaataaaaaacatttattttcattgcaatgatgtatttaaattatttctgaatattttactaaaaagggaatgtgggaggtcagtgcatttaaaacataaagaaatgaagagctagttcaaaccttgggaaaatacactatatcttaaa

SEQ ID NO: 14 - DNA, 222 bp, Artificial Sequence
  SV40 late polyA
cagacatgataagatacattgatgagtttggacaaaccacaactagaatgcagtgaaaaaaatgctttatttgtgaaatttgtgatgctattgctttatttgtaaccattataagctgcaataaacaagttaacaacaacaattgcattcattttatgtttcaggttcagggggaggtgtgggaggttttttaaagcaagtaaaacctctacaaatgtggta

SEQ ID NO: 15 - DNA, 197 bp, Artificial Sequence
  SV40 promoter
tgcatctcaattagtcagcaaccatagtcccgcccctaactccgcccatcccgcccctaactccgcccagttccgcccattctccgccccatcgctgactaattttttttatttatgcagaggccgaggccgcctcggcctctgagctattccagaagtagtgaggaggcttttttggaggcctaggcttttgcaaa

SEQ ID NO: 16 - DNA, 538 bp, Artificial Sequence
  human CMV immediate-early enhancer/promoter
ggagttccgcgttacataacttacggtaaatggcccgcctggctgaccgcccaacgacccccgcccattgacgtcaataatgacgtatgttcccatagtaacgccaatagggactttccattgacgtcaatgggtggagtatttacggtaaactgcccacttggcagtacatcaagtgtatcatatgccaagtacgccccctattgacgtcaatgacggtaaatggcccgcctggcattatgcccagtacatgaccttatgggactttcctacttggcagtacatctacgtattagtcatcgctattaccatggtgatgcggttttggcagtacatcaatgggcgtggatagcggtttgactcacggggatttccaagtctccaccccattgacgtcaatgggagtttgttttggcaccaaaatcaacgggactttccaaaatgtcgtaacaactccgccccattgacgcaaatgggcggtaggcgtgtacggtgggaggtctatataagcagagctcgtttagtgaaccgtcagatc

SEQ ID NO: 17 - DNA, 366 bp, Artificial Sequence
  TPL
ctcttccgcatcgctgtctgcgagggccagctgttggggtgagtactccctctcaaaagcgggcatgacttctgcgctaagattgtcagtttccaaaaacgaggaggatttgatattcacctggcccgcggtgatgcctttgagggtggccgcgtccatctggtcagaaaagacaatctttttgttgtcaagcttccttgatgatgtcatacttatcctgtcccttttttttccacagctcgcggttgaggacaaactcttcgcggtctttccagtactcttggatcggaaacccgtcggcctccgaacggtactccgccaccgagggacctgagcgagtccgcatcgaccggatcggaaaacctc

SEQ ID NO: 18 - DNA, 528 bp, Artificial Sequence
  Human CMV promoter, derived from GenBank X17403.1
gttacataacttacggtaaatggcccgcctggctgaccgcccaacgacccccgcccattgacgtcaataatgacgtatgttcccatagtaacgccaatagggactttccattgacgtcaatgggtggagtatttacggtaaactgcccacttggcagtacatcaagtgtatcatatgccaagtacgccccctattgacgtcaatgacggtaaatggcccgcctggcattatgcccagtacatgaccttatgggactttcctacttggcagtacatctacgtattagtcatcgctattaccatggtgatgcggttttggcagtacatcaatgggcgtggatagcggtttgactcacggggatttccaagtctccaccccattgacgtcaatgggagtttgttttggcaccaaaatcaacgggactttccaaaatgtcgtaacaactccgccccattgacgcaaatgggcggtaggcgtgtacggtgggaggtctatataagcagagctcgtttagtgaaccgtcagatc

SEQ ID NO: 19 - DNA, 589 bp, Artificial Sequence
  Bacterial replication origin
tttccataggctccgcccccctgacgagcatcacaaaaatcgacgctcaagtcagaggtggcgaaacccgacaggactataaagataccaggcgtttccccctggaagctccctcgtgcgctctcctgttccgaccctgccgcttaccggatacctgtccgcctttctcccttcgggaagcgtggcgctttctcatagctcacgctgtaggtatctcagttcggtgtaggtcgttcgctccaagctgggctgtgtgcacgaaccccccgttcagcccgaccgctgcgccttatccggtaactatcgtcttgagtccaacccggtaagacacgacttatcgccactggcagcagccactggtaacaggattagcagagcgaggtatgtaggcggtgctacagagttcttgaagtggtggcctaactacggctacactagaaggacagtatttggtatctgcgctctgctgaagccagttaccttcggaaaaagagttggtagctcttgatccggcaaacaaaccaccgctggtagcggtggtttttttgtttgcaagcagcagattacgcgcagaaaaaaaggatctcaa

SEQ ID NO: 20 - DNA, 861 bp, Artificial Sequence
  Ampicillin resistance gene
ttaccaatgcttaatcagtgaggcacctatctcagcgatctgtctatttcgttcatccatagttgcctgactccccgtcgtgtagataactacgatacgggagggcttaccatctggccccagtgctgcaatgataccgcgagacccacgctcaccggctccagatttatcagcaataaaccagccagccggaagggccgagcgcagaagtggtcctgcaactttatccgcctccatccagtctattaattgttgccgggaagctagagtaagtagttcgccagttaatagtttgcgcaacgttgttgccattgctacaggcatcgtggtgtcacgctcgtcgtttggtatggcttcattcagctccggttcccaacgatcaaggcgagttacatgatcccccatgttgtgcaaaaaagcggttagctccttcggtcctccgatcgttgtcagaagtaagttggccgcagtgttatcactcatggttatggcagcactgcataattctcttactgtcatgccatccgtaagatgcttttctgtgactggtgagtactcaaccaagtcattctgagaatagtgtatgcggcgaccgagttgctcttgcccggcgtcaatacgggataataccgcgccacatagcagaactttaaaagtgctcatcattggaaaacgttcttcggggcgaaaactctcaaggatcttaccgctgttgagatccagttcgatgtaacccactcgtgcacccaactgatcttcagcatcttttactttcaccagcgtttctgggtgagcaaaaacaggaaggcaaaatgccgcaaaaaagggaataagggcgacacggaaatgttgaatactcat

SEQ ID NO: 21 - DNA, 1122 bp, Artificial Sequence
  GS gene
atggccacctcagcaagttcccacttgaacaaaaacatcaagcaaatgtacttgtgcctgccccagggtgagaaagtccaagccatgtatatctgggttgatggtactggagaaggactgcgctgcaaaacccgcaccctggactgtgagcccaagtgtgtagaagagttacctgagtggaattttgatggctctagtacctttcagtctgagggctccaacagtgacatgtatctcagccctgttgccatgtttcgggaccccttccgcagagatcccaacaagctggtgttctgtgaagttttcaagtacaaccggaagcctgcagagaccaatttaaggcactcgtgtaaacggataatggacatggtgagcaaccagcacccctggtttggaatggaacaggagtatactctgatgggaacagatgggcacccttttggttggccttccaatggctttcctgggccccaaggtccgtattactgtggtgtgggcgcagacaaagcctatggcagggatatcgtggaggctcactaccgcgcctgcttgtatgctggggtcaagattacaggaacaaatgctgaggtcatgcctgcccagtgggagttccaaataggaccctgtgaaggaatccgcatgggagatcatctctgggtggcccgtttcatcttgcatcgagtatgtgaagactttggggtaatagcaacctttgaccccaagcccattcctgggaactggaatggtgcaggctgccataccaactttagcaccaaggccatgcgggaggagaatggtctgaagcacatcgaggaggccatcgagaaactaagcaagcggcaccggtaccacattcgagcctacgatcccaaggggggcctggacaatgcccgtcgtctgactgggttccacgaaacgtccaacatcaacgacttttctgctggtgtcgccaatcgcagtgccagcatccgcattccccggactgtcggccaggagaagaaaggttactttgaagaccgccgcccctctgccaattgtgacccctttgcagtgacagaagccatcgtccgcacatgccttctcaatgagactggcgacgagcccttccaatacaaaaactaa

SEQ ID NO: 22 - DNA, 237 bp, Artificial Sequence
  SV40 enhancer
gctgtggaatgtgtgtcagttagggtgtggaaagtccccaggctccccagcaggcagaagtatgcaaagcatgcatctcaattagtcagcaaccaggtgtggaaagtccccaggctccccagcaggcagaagtatgcaaagcatgcatctcaattagtcagcaaccatagtcccgcccctaactccgcccatcccgcccctaactccgcccagttccgcccattctccgctccatcg

SEQ ID NO: 23 - DNA, 570 bp, Artificial Sequence
  IRES-4
cccctaacgttactggccgaagccgcttggaataaggccggtgtgcgtttgtctatatgttattttccaccatattgccgtcttttggcaatgtgagggcccggaaacctggccctgtcttcttgacgagcattcctaggggtctttcccctctcgccaaaggaatgcaaggtctgttgaatgtcgtgaaggaagcagttcctctggaagcttcttgaagacaaacaacgtctgtagcgaccctttgcaggcagcggaaccccccacctggcgacaggtgcctctgcggccaaaagccacgtgtataagatacacctgcaaaggcggcacaaccccagtgccacgttgtgagttggatagttgtggaaagagtcaaatggctctcctcaagcgtattcaacaaggggctgaaggatgcccagaaggtaccccattgtatgggatctgatctggggcctcggtgcacatgctttacatgtgtttagtcgaggttaaaaaaacgtctaggccccccgaaccacggggacgtggttttcctttgaaaaacacgatgataatatggccacaacc

SEQ ID NO: 24 - DNA, 557 bp, Artificial Sequence
  IRES-5
cccctaacgttactggccgaagccgcttggaataaggccggtgtgcgtttgtctatatgttattttccaccatattgccgtcttttggcaatgtgagggcccggaaacctggccctgtcttcttgacgagcattcctaggggtctttcccctctcgccaaaggaatgcaaggtctgttgaatgtcgtgaaggaagcagttcctctggaagcttcttgaagacaaacaacgtctgtagcgaccctttgcaggcagcggaaccccccacctggcgacaggtgcctctgcggccaaaagccacgtgtataagatacacctgcaaaggcggcacaaccccagtgccacgttgtgagttggatagttgtggaaagagtcaaatggctctcctcaagcgtattcaacaaggggctgaaggatgcccagaaggtaccccattgtatgggatctgatctggggcctcggtgcacatgctttacatgtgtttagtcgaggttaaaaaaacgtctaggccccccgaaccacggggacgtggttttcctttgaaaaacacgatgataa

SEQ ID NO: 25 - DNA, 550 bp, Artificial Sequence
  IRES-6
cccctaacgttactggccgaagccgcttggaataaggccggtgtgcgtttgtctatatgttattttccaccatattgccgtcttttggcaatgtgagggcccggaaacctggccctgtcttcttgacgagcattcctaggggtctttcccctctcgccaaaggaatgcaaggtctgttgaatgtcgtgaaggaagcagttcctctggaagcttcttgaagacaaacaacgtctgtagcgaccctttgcaggcagcggaaccccccacctggcgacaggtgcctctgcggccaaaagccacgtgtataagatacacctgcaaaggcggcacaaccccagtgccacgttgtgagttggatagttgtggaaagagtcaaatggctctcctcaagcgtattcaacaaggggctgaaggatgcccagaaggtaccccattgtatgggatctgatctggggcctcggtgcacatgctttacatgtgtttagtcgaggttaaaaaaacgtctaggccccccgaaccacggggacgtggttttcctttgaaaaacacg

SEQ ID NO: 26 - DNA, 10754 bp, Artificial Sequence
  pCLD13
ccctagaaagataatcatattgtgacgtacgttaaagataatcatgcgtaaaattgacgcatgtgttttatcggtctgtatatcgaggtttatttattaatttgaatagatattaagttttattatatttacacttacatactaataataaattcaacaaacaatttatttatgtttatttatttattaaaaaaaaacaaaaactcaaaatttcttctataaagtaacaaaacttttatcgaatttgcagcccgggactagctagagggacagcccccccccaaagcccccagggatgtaattacgtccctcccccgctagggggcagcagcgagccgcccggggctccgctccggtccggcgctccccccgcatccccgagccggcagcgtgcggggacagcccgggcacggggaaggtggcacgggatcgctttcctctgaacgcttctcgctgctctttgagcctgcagacacctggggggatacggggaaaacttaagatccgaccggacgcgtactgagagcgctattctgaacttttcttttgttcccttcccttctaccacaccctaattgtaatccattttaatttcctggtcacagtcctgtctctccttccattgtaccttgcccttttctaaagagcgactgcaaagtatgtttgcgtaggtgaggatctaaaactttatgaggtacgaacatcacagaattactttgtaatttcagtttattgtaggcttggctttttggggagggtttacgtcttagacctcttagtgcttctttgtttcatggtgttctaacttcgaagcatctctgtagctttaatggattccttttctgaaagctttgctctctttcttccccctcggctttctcttaggcaagagggctaactgtaaagtaaggcttactgccttgtgtttccaaatgtgtccgaagaggaagtgtcttctgtgaatcctgttatgcatgaataacaggaaatagaaagaaattcactttcattattataaaagtaatatgttcgtttaaaaaattctaatgaagagctggagatgcaacccaggggtagagcacacactcagcatgcaggaggccctgggtccaatcttggaatctcctctcagttaacctgatctctagctgattagtagtgagtgcaagcccactttcctcttctgcctcattgctcagtgataacagctgttaaactttgtcttattctaaaactacctctgtgcaaatgctagcacaataatatatatcatatgcacatgattttttttttatcttgaaaagtaagtcagtatagctacaaagttcacttggcattgtcaacatttcacaggcgtaatattcctcctctagtactgtcctcttcattctttgtgaccaagtttggagagagtgcacaaatgccagggaggtttgtgggaaggtttctcatgttctggtaaggcgagtaagaaaatagtctcatgcaggtgaaatgagtgctatgcagtatatattataccagagaacagcaaatgaccaaattcacactgaactagttcagtaaaattggctttgtcaaagctttccttgcttaaaatgtaattccctgtcatcctagttctggtctggattcttttcctggagtcttgacttccagattccctgtggacttttgtttgagtttcaagcttttgaaatatagaaacctatctaacttaacaaacttgggagagaaaagactccagaacaactgaaaacagaccaggctaaatgaatagactttattcctctcttcttacctgcagttttcagatatgcagagttggagcggatcttagaggttgattcattcatgcctgaagaaaacacattttatagaccctgtgcccaagttcgtggtggacatcaccctttatttactaattgcactacataacaggcattttagaagactgctccagtcagagaccccgccttagaggaatctgtaaaccctgaactcctatcactcatgagcactagttatgtttggaatgccgtattaaaacaaaagttacatttctaaacttaaaattttctagcacagagacagtgggagtagctaactttgatagacatttttctactaaaagtctttctaagtacataatcttctgtaagttggaaaacagcaaaatagaacgtctcctacgtagttaatctttttgcataatttgcacatgtaggagttattagtatacgggtaagttttcactttttcccccaactggagtgtcttgtggctgggtttgaaaaagggaacgggaggccgctggaggggattggtaaatgagataaaacaccactcattcaactcagtgactcagcatttaaattttccataaaaggattaaaggaaaattaaacaaattcttaaagccaagactctggagaaacttgttggtgtgctttagttttcactgttatgactcatgaatttatgcataaattagtacatttataaaaacatagcctttttagagttttctgtttggctaaagtgccattgttagcatttggaattacctttttatgtcttatattttttccaaataaaaataaatgtttctgctgtcttactactgaaactacgttgtgagcactttaaatttctcaaagcagtttcgcctgttatacttggcgcttagtcatcgtcgtacacaacaggacctgattaagaaggctgtgctgcctctaagccgggctagattgtagccactagcaaccaggctgcaataatttccctttgatgacatcatccactgtggaagaacccagttgcttcagccagtcgaactatacagttccaacctcatcaaatatggcatctcccttgcctgctatagcagggggaggaaaaaatgccaccatctttttaatctagcaagcttctcttttcttcatctttttttttttcttttaaaaaaattctgatcatggatgcttcttccgatccctatttgccttatgacgggggaggagacaatatccccttgagggaattacataaaagaggtaagagcatccccttgctctgaatcctctgttggttgttgtgcatgcggctgggcggttctggggacaggctgtctgttgtcctcttgctgcaatgtgctgcttagttgccctgccttgttgctgtgggagaatgcgaccttcccagcagggctggccctccctgattgtttgctctgtgcagattagccctgcttcagatcacatagggctgcagactccatcttctgtgtgaaaatgctttcggtttgattgcagaaataagctgcctttacagccagctaaagtcctggtggttggttggcacctgcaaagtagtatttttgtacctctggaaacttatattttctttacacagcaatatcaagtgccggtatgccattctgttttggctgctgccaattaccatgtagactttgcaccacagagtaatagtaaaagctcctagctgcattttataacatttaaaaatagcaggaaagaagaattatttttgatttaacatgtttttgtcatttaacgtcttaactgattgacatactatattgtctgtctcgtgggtatcttgtacaacttgataggataaagcaatttagtttttttttttttttttaaatacatccagaatgtaagtcgtcagtagttttcgaacagataagtaatggtgttaatcttttggcaggctttgccttggtctccttaaagctaattaggtgttacttaattaaactgctcttttgctcattttcttaaattatttttttaaaagatagttggcatttgctgttctagaaataaacttcaagaaacattctttagccagatgacttcatgtatgagccatgttagtttgaattatttgcttggtgttataaactttatggtttaataccaacttttattatgtttacaaggtaaataaggaaaatttcaagtacattttgtatcctgagaacaaatttaagttccatagaatttaggaattacaatgtattcaacagatacttacttgtcatactgtgcctgcaaaacaataattagactctgaacaggtgcaacaattttctgtagaattagacaagtcttcttttggcaggtgttactaagtaggccatttcccaaggaacagggaatttgccaggcttttgtggtggagagaatagaatgaataaatgctgtggggagtaaagagcttgtcagaagatgattagttctgtggcaccaaaaccaagagatcagttttcctgtgagaagtaaaggaagcattgtagaaaaatagatgtgttgaagtctaccggtggagttccgcgttacataacttacggtaaatggcccgcctggctgaccgcccaacgacccccgcccattgacgtcaataatgacgtatgttcccatagtaacgccaatagggactttccattgacgtcaatgggtggagtatttacggtaaactgcccacttggcagtacatcaagtgtatcatatgccaagtacgccccctattgacgtcaatgacggtaaatggcccgcctggcattatgcccagtacatgaccttatgggactttcctacttggcagtacatctacgtattagtcatcgctattaccattgtgatgcggttttggcagtacatcaatgggcgtggatagcggtttgactcacggggatttccaagtctccaccccattgacgtcaatgggagtttgttttggcaccaaaatcaacgggactttccaaaatgtcgtaacaactccgccccattgacgcaaatgggcggtaggcgtgtacggtgggaggtctatataagcagagctcgtttagtgaaccgtcagatctacctcttccgcatcgctgtctgcgagggccagctgttggggtgagtactccctctcaaaagcgggcatgacttctgcgctaagattgtcagtttccaaaaacgaggaggatttgatattcacctggcccgcggtgatgcctttgagggtggccgcgtccatctggtcagaaaagacaatctttttgttgtcaagcttccttgatgatgtcatacttatcctgtcccttttttttccacagctcgcggttgaggacaaactcttcgcggtctttccagtactcttggatcggaaacccgtcggcctccgaacggtactccgccaccgagggacctgagcgagtccgcatcgaccggatcggaaaacctcggatccgaattcatagataactgatccagtgcccctaacgttactggccgaagccgcttggaataaggccggtgtgcgtttgtctatatgttattttccaccatattgccgtcttttggcaatgtgagggcccggaaacctggccctgtcttcttgacgagcattcctaggggtctttcccctctcgccaaaggaatgcaaggtctgttgaatgtcgtgaaggaagcagttcctctggaagcttcttgaagacaaacaacgtctgtagcgaccctttgcaggcagcggaaccccccacctggcgacaggtgcctctgcggccaaaagccacgtgtataagatacacctgcaaaggcggcacaaccccagtgccacgttgtgagttggatagttgtggaaagagtcaaatggctctcctcaagcgtattcaacaaggggctgaaggatgcccagaaggtaccccattgtatgggatctgatctggggcctcggtgcacatgctttacatgtgtttagtcgaggttaaaaaacgtctaggccccccgaaccacggggacgtggttttcctttgaaaaacacgatgataaatggccacctcagcaagttcccacttgaacaaaaacatcaagcaaatgtacttgtgcctgccccagggtgagaaagtccaagccatgtatatctgggttgatggtactggagaaggactgcgctgcaaaacccgcaccctggactgtgagcccaagtgtgtagaagagttacctgagtggaattttgatggctctagtacctttcagtctgagggctccaacagtgacatgtatctcagccctgttgccatgtttcgggaccccttccgcagagatcccaacaagctggtgttctgtgaagttttcaagtacaaccggaagcctgcagagaccaatttaaggcactcgtgtaaacggataatggacatggtgagcaaccagcacccctggtttggaatggaacaggagtatactctgatgggaacagatgggcacccttttggttggccttccaatggctttcctgggccccaaggtccgtattactgtggtgtgggcgcagacaaagcctatggcagggatatcgtggaggctcactaccgcgcctgcttgtatgctggggtcaagattacaggaacaaatgctgaggtcatgcctgcccagtgggagttccaaataggaccctgtgaaggaatccgcatgggagatcatctctgggtggcccgtttcatcttgcatcgagtatgtgaagactttggggtaatagcaacctttgaccccaagcccattcctgggaactggaatggtgcaggctgccataccaactttagcaccaaggccatgcgggaggagaatggtctgaagcacatcgaggaggccatcgagaaactaagcaagcggcaccggtaccacattcgagcctacgatcccaaggggggcctggacaatgcccgtcgtctgactgggttccacgaaacgtccaacatcaacgacttttctgctggtgtcgccaatcgcagtgccagcatccgcattccccggactgtcggccaggagaagaaaggttactttgaagaccgccgcccctctgccaattgtgacccctttgcagtgacagaagccatcgtccgcacatgccttctcaatgagactggcgacgagcccttccaatacaaaaactaatctagatccccctcgctttcttgctgtccaatttctattaaaggttcctttgttccctaagtccaactactaaactgggggatattatgaagggccttgagcatctggattctgcctaataaaaaacatttattttcattgcaatgatgtatttaaattatttctgaatattttactaaaaagggaatgtgggaggtcagtgcatttaaaacataaagaaatgaagagggggatcttcgcgatactgcatcgatgagggacagcccccccccaaagcccccagggatgtaattacgtccctcccccgctagggggcagcagcgagccgcccggggctccgctccggtccggcgctccccccgcatccccgagccggcagcgtgcggggacagcccgggcacggggaaggtggcacgggatcgctttcctctgaacgcttctcgctgctctttgagcctgcagacacctggggggatacggggaaaatagacaccgcggtggagctccagcttttgttccctttagtgagggttaattagttcttaatacgactcactatagggcgaattggctaccgggccgcccatcgagggtatcataagcttatatctataacaagaaaatatatatataataagttatcacgtaagtagaacatgaaataacaatataattatcgtatgagttaaatcttaaaagtcacgtaaaagataatcatgcgtcattttgactcacgcggtcgttatagttcaaaatcagtgacacttaccgcattgacaagcacgcctcacgggagctccaagcggcgactgagatgtcctaaatgcacagcgacggattcgcgctatttagaaagagagagcaatatttcaagaatgcatgcgtcaattttacgcagactatctttctagggttaaatcgatagatgcgatcctgcaggtctccctatagtgagtcgtattaatttcgataagccagctgcattaatgaatcggccaacgcgcggggagaggcggtttgcgtattgggcgctcttccgcttcctcgctcactgactcgctgcgctcggtcgttcggctgcggcgagcggtatcagctcactcaaaggcggtaatacggttatccacagaatcaggggataacgcaggaaagaacatgtgagcaaaaggccagcaaaaggccaggaaccgtaaaaaggccgcgttgctggcgtttttccataggctccgcccccctgacgagcatcacaaaaatcgacgctcaagtcagaggtggcgaaacccgacaggactataaagataccaggcgtttccccctggaagctccctcgtgcgctctcctgttccgaccctgccgcttaccggatacctgtccgcctttctcccttcgggaagcgtggcgctttctcatagctcacgctgtaggtatctcagttcggtgtaggtcgttcgctccaagctgggctgtgtgcacgaaccccccgttcagcccgaccgctgcgccttatccggtaactatcgtcttgagtccaacccggtaagacacgacttatcgccactggcagcagccactggtaacaggattagcagagcgaggtatgtaggcggtgctacagagttcttgaagtggtggcctaactacggctacactagaaggacagtatttggtatctgcgctctgctgaagccagttaccttcggaaaaagagttggtagctcttgatccggcaaacaaaccaccgctggtagcggtggtttttttgtttgcaagcagcagattacgcgcagaaaaaaaggatctcaagaagatcctttgatcttttctacggggtctgacgctcagtggaacgaaaactcacgttaagggattttggtcatgagattatcaaaaaggatcttcacctagatccttttaaattaaaaatgaagttttaaatcaatctaaagtatatatgagtaaacttggtctgacagttaccaatgcttaatcagtgaggcacctatctcagcgatctgtctatttcgttcatccatagttgcctgactccccgtcgtgtagataactacgatacgggagggcttaccatctggccccagtgctgcaatgataccgcgagacccacgctcaccggctccagatttatcagcaataaaccagccagccggaagggccgagcgcagaagtggtcctgcaactttatccgcctccatccagtctattaattgttgccgggaagctagagtaagtagttcgccagttaatagtttgcgcaacgttgttgccattgctacaggcatcgtggtgtcacgctcgtcgtttggtatggcttcattcagctccggttcccaacgatcaaggcgagttacatgatcccccatgttgtgcaaaaaagcggttagctccttcggtcctccgatcgttgtcagaagtaagttggccgcagtgttatcactcatggttatggcagcactgcataattctcttactgtcatgccatccgtaagatgcttttctgtgactggtgagtactcaaccaagtcattctgagaatagtgtatgcggcgaccgagttgctcttgcccggcgtcaatacgggataataccgcgccacatagcagaactttaaaagtgctcatcattggaaaacgttcttcggggcgaaaactctcaaggatcttaccgctgttgagatccagttcgatgtaacccactcgtgcacccaactgatcttcagcatcttttactttcaccagcgtttctgggtgagcaaaaacaggaaggcaaaatgccgcaaaaaagggaataagggcgacacggaaatgttgaatactcatactcttcctttttcaatattattgaagcatttatcagggttattgtctcatgagcggatacatatttgaatgtatttagaaaaataaacaaataggggttccgcgcacatttccccgaaaagtgccacctgacgtctaagaaaccattattatcatgacattaacctataaaaataggcgtatcacgaggccctttcgtctcgcgcgtttcggtgatgacggtgaaaacctctgacacatgcagctcccggagacggtcacagcttgtctgtaagcggatgccgggagcagacaagcccgtcagggcgcgtcagcgggtgttggcgggtgtcggggctggcttaactatgcggcatcagagcagattgtactgagagtgcaccatatcgacgctctcccttatgcgactcctgcattaggaagcagcccagtagtaggttgaggccgttgagcaccgccgccgcaaggaatggtgcatgcaaggagatggcgcccaacagtcccccggccacggggcctgccaccatacccacgccgaaacaagcgctcatgagcccgaagtggcgagcccgatcttccccatcggtgatgtcggcgatataggcgccagcaaccgcacctgtggcgccggtgatgccggccacgatgcgtccggcgtagaggatctggctagcgatgaccctgctgattggttcgctgaccatttccggggtgcggaacggcgttaccagaaactcagaaggttcgtccaaccaaaccgactctgacggcagtttacgagagagatgatagggtctgcttcagtaagccagatgctacacaattaggcttgtacatattgtcgttagaacgcggctacaattaatacataaccttatgtatcatacacatacgatttaggtgacactatagaatacacctgcaggacgtcccaatgatcttaagttaa

SEQ ID NO: 27 - DNA, 10768 bp, Artificial Sequence
  pCLD15
ccctagaaagataatcatattgtgacgtacgttaaagataatcatgcgtaaaattgacgcatgtgttttatcggtctgtatatcgaggtttatttattaatttgaatagatattaagttttattatatttacacttacatactaataataaattcaacaaacaatttatttatgtttatttatttattaaaaaaaaacaaaaactcaaaatttcttctataaagtaacaaaacttttatcgaatttgcagcccgggactagctagagggacagcccccccccaaagcccccagggatgtaattacgtccctcccccgctagggggcagcagcgagccgcccggggctccgctccggtccggcgctccccccgcatccccgagccggcagcgtgcggggacagcccgggcacggggaaggtggcacgggatcgctttcctctgaacgcttctcgctgctctttgagcctgcagacacctggggggatacggggaaaacttaagatccgaccggacgcgtactgagagcgctattctgaacttttcttttgttcccttcccttctaccacaccctaattgtaatccattttaatttcctggtcacagtcctgtctctccttccattgtaccttgcccttttctaaagagcgactgcaaagtatgtttgcgtaggtgaggatctaaaactttatgaggtacgaacatcacagaattactttgtaatttcagtttattgtaggcttggctttttggggagggtttacgtcttagacctcttagtgcttctttgtttcatggtgttctaacttcgaagcatctctgtagctttaatggattccttttctgaaagctttgctctctttcttccccctcggctttctcttaggcaagagggctaactgtaaagtaaggcttactgccttgtgtttccaaatgtgtccgaagaggaagtgtcttctgtgaatcctgttatgcatgaataacaggaaatagaaagaaattcactttcattattataaaagtaatatgttcgtttaaaaaattctaatgaagagctggagatgcaacccaggggtagagcacacactcagcatgcaggaggccctgggtccaatcttggaatctcctctcagttaacctgatctctagctgattagtagtgagtgcaagcccactttcctcttctgcctcattgctcagtgataacagctgttaaactttgtcttattctaaaactacctctgtgcaaatgctagcacaataatatatatcatatgcacatgattttttttttatcttgaaaagtaagtcagtatagctacaaagttcacttggcattgtcaacatttcacaggcgtaatattcctcctctagtactgtcctcttcattctttgtgaccaagtttggagagagtgcacaaatgccagggaggtttgtgggaaggtttctcatgttctggtaaggcgagtaagaaaatagtctcatgcaggtgaaatgagtgctatgcagtatatattataccagagaacagcaaatgaccaaattcacactgaactagttcagtaaaattggctttgtcaaagctttccttgcttaaaatgtaattccctgtcatcctagttctggtctggattcttttcctggagtcttgacttccagattccctgtggacttttgtttgagtttcaagcttttgaaatatagaaacctatctaacttaacaaacttgggagagaaaagactccagaacaactgaaaacagaccaggctaaatgaatagactttattcctctcttcttacctgcagttttcagatatgcagagttggagcggatcttagaggttgattcattcatgcctgaagaaaacacattttatagaccctgtgcccaagttcgtggtggacatcaccctttatttactaattgcactacataacaggcattttagaagactgctccagtcagagaccccgccttagaggaatctgtaaaccctgaactcctatcactcatgagcactagttatgtttggaatgccgtattaaaacaaaagttacatttctaaacttaaaattttctagcacagagacagtgggagtagctaactttgatagacatttttctactaaaagtctttctaagtacataatcttctgtaagttggaaaacagcaaaatagaacgtctcctacgtagttaatctttttgcataatttgcacatgtaggagttattagtatacgggtaagttttcactttttcccccaactggagtgtcttgtggctgggtttgaaaaagggaacgggaggccgctggaggggattggtaaatgagataaaacaccactcattcaactcagtgactcagcatttaaattttccataaaaggattaaaggaaaattaaacaaattcttaaagccaagactctggagaaacttgttggtgtgctttagttttcactgttatgactcatgaatttatgcataaattagtacatttataaaaacatagcctttttagagttttctgtttggctaaagtgccattgttagcatttggaattacctttttatgtcttatattttttccaaataaaaataaatgtttctgctgtcttactactgaaactacgttgtgagcactttaaatttctcaaagcagtttcgcctgttatacttggcgcttagtcatcgtcgtacacaacaggacctgattaagaaggctgtgctgcctctaagccgggctagattgtagccactagcaaccaggctgcaataatttccctttgatgacatcatccactgtggaagaacccagttgcttcagccagtcgaactatacagttccaacctcatcaaatatggcatctcccttgcctgctatagcagggggaggaaaaaatgccaccatctttttaatctagcaagcttctcttttcttcatctttttttttttcttttaaaaaaattctgatcatggatgcttcttccgatccctatttgccttatgacgggggaggagacaatatccccttgagggaattacataaaagaggtaagagcatccccttgctctgaatcctctgttggttgttgtgcatgcggctgggcggttctggggacaggctgtctgttgtcctcttgctgcaatgtgctgcttagttgccctgccttgttgctgtgggagaatgcgaccttcccagcagggctggccctccctgattgtttgctctgtgcagattagccctgcttcagatcacatagggctgcagactccatcttctgtgtgaaaatgctttcggtttgattgcagaaataagctgcctttacagccagctaaagtcctggtggttggttggcacctgcaaagtagtatttttgtacctctggaaacttatattttctttacacagcaatatcaagtgccggtatgccattctgttttggctgctgccaattaccatgtagactttgcaccacagagtaatagtaaaagctcctagctgcattttataacatttaaaaatagcaggaaagaagaattatttttgatttaacatgtttttgtcatttaacgtcttaactgattgacatactatattgtctgtctcgtgggtatcttgtacaacttgataggataaagcaatttagtttttttttttttttttaaatacatccagaatgtaagtcgtcagtagttttcgaacagataagtaatggtgttaatcttttggcaggctttgccttggtctccttaaagctaattaggtgttacttaattaaactgctcttttgctcattttcttaaattatttttttaaaagatagttggcatttgctgttctagaaataaacttcaagaaacattctttagccagatgacttcatgtatgagccatgttagtttgaattatttgcttggtgttataaactttatggtttaataccaacttttattatgtttacaaggtaaataaggaaaatttcaagtacattttgtatcctgagaacaaatttaagttccatagaatttaggaattacaatgtattcaacagatacttacttgtcatactgtgcctgcaaaacaataattagactctgaacaggtgcaacaattttctgtagaattagacaagtcttcttttggcaggtgttactaagtaggccatttcccaaggaacagggaatttgccaggcttttgtggtggagagaatagaatgaataaatgctgtggggagtaaagagcttgtcagaagatgattagttctgtggcaccaaaaccaagagatcagttttcctgtgagaagtaaaggaagcattgtagaaaaatagatgtgttgaagtctaccggtggagttccgcgttacataacttacggtaaatggcccgcctggctgaccgcccaacgacccccgcccattgacgtcaataatgacgtatgttcccatagtaacgccaatagggactttccattgacgtcaatgggtggagtatttacggtaaactgcccacttggcagtacatcaagtgtatcatatgccaagtacgccccctattgacgtcaatgacggtaaatggcccgcctggcattatgcccagtacatgaccttatgggactttcctacttggcagtacatctacgtattagtcatcgctattaccattgtgatgcggttttggcagtacatcaatgggcgtggatagcggtttgactcacggggatttccaagtctccaccccattgacgtcaatgggagtttgttttggcaccaaaatcaacgggactttccaaaatgtcgtaacaactccgccccattgacgcaaatgggcggtaggcgtgtacggtgggaggtctatataagcagagctcgtttagtgaaccgtcagatctacctcttccgcatcgctgtctgcgagggccagctgttggggtgagtactccctctcaaaagcgggcatgacttctgcgctaagattgtcagtttccaaaaacgaggaggatttgatattcacctggcccgcggtgatgcctttgagggtggccgcgtccatctggtcagaaaagacaatctttttgttgtcaagcttccttgatgatgtcatacttatcctgtcccttttttttccacagctcgcggttgaggacaaactcttcgcggtctttccagtactcttggatcggaaacccgtcggcctccgaacggtactccgccaccgagggacctgagcgagtccgcatcgaccggatcggaaaacctcggatccgaattcatagataactgatccagtgcccctaacgttactggccgaagccgcttggaataaggccggtgtgcgtttgtctatatgttattttccaccatattgccgtcttttggcaatgtgagggcccggaaacctggccctgtcttcttgacgagcattcctaggggtctttcccctctcgccaaaggaatgcaaggtctgttgaatgtcgtgaaggaagcagttcctctggaagcttcttgaagacaaacaacgtctgtagcgaccctttgcaggcagcggaaccccccacctggcgacaggtgcctctgcggccaaaagccacgtgtataagatacacctgcaaaggcggcacaaccccagtgccacgttgtgagttggatagttgtggaaagagtcaaatggctctcctcaagcgtattcaacaaggggctgaaggatgcccagaaggtaccccattgtatgggatctgatctggggcctcggtgcacatgctttacatgtgtttagtcgaggttaaaaaaacgtctaggccccccgaaccacggggacgtggttttcctttgaaaaacacgatgataatatggccacaaccatggccacctcagcaagttcccacttgaacaaaaacatcaagcaaatgtacttgtgcctgccccagggtgagaaagtccaagccatgtatatctgggttgatggtactggagaaggactgcgctgcaaaacccgcaccctggactgtgagcccaagtgtgtagaagagttacctgagtggaattttgatggctctagtacctttcagtctgagggctccaacagtgacatgtatctcagccctgttgccatgtttcgggaccccttccgcagagatcccaacaagctggtgttctgtgaagttttcaagtacaaccggaagcctgcagagaccaatttaaggcactcgtgtaaacggataatggacatggtgagcaaccagcacccctggtttggaatggaacaggagtatactctgatgggaacagatgggcacccttttggttggccttccaatggctttcctgggccccaaggtccgtattactgtggtgtgggcgcagacaaagcctatggcagggatatcgtggaggctcactaccgcgcctgcttgtatgctggggtcaagattacaggaacaaatgctgaggtcatgcctgcccagtgggagttccaaataggaccctgtgaaggaatccgcatgggagatcatctctgggtggcccgtttcatcttgcatcgagtatgtgaagactttggggtaatagcaacctttgaccccaagcccattcctgggaactggaatggtgcaggctgccataccaactttagcaccaaggccatgcgggaggagaatggtctgaagcacatcgaggaggccatcgagaaactaagcaagcggcaccggtaccacattcgagcctacgatcccaaggggggcctggacaatgcccgtcgtctgactgggttccacgaaacgtccaacatcaacgacttttctgctggtgtcgccaatcgcagtgccagcatccgcattccccggactgtcggccaggagaagaaaggttactttgaagaccgccgcccctctgccaattgtgacccctttgcagtgacagaagccatcgtccgcacatgccttctcaatgagactggcgacgagcccttccaatacaaaaactaatctagatccccctcgctttcttgctgtccaatttctattaaaggttcctttgttccctaagtccaactactaaactgggggatattatgaagggccttgagcatctggattctgcctaataaaaaacatttattttcattgcaatgatgtatttaaattatttctgaatattttactaaaaagggaatgtgggaggtcagtgcatttaaaacataaagaaatgaagagggggatcttcgcgatactgcatcgatgagggacagcccccccccaaagcccccagggatgtaattacgtccctcccccgctagggggcagcagcgagccgcccggggctccgctccggtccggcgctccccccgcatccccgagccggcagcgtgcggggacagcccgggcacggggaaggtggcacgggatcgctttcctctgaacgcttctcgctgctctttgagcctgcagacacctggggggatacggggaaaatagacaccgcggtggagctccagcttttgttccctttagtgagggttaattagttcttaatacgactcactatagggcgaattggctaccgggccgcccatcgagggtatcataagcttatatctataacaagaaaatatatatataataagttatcacgtaagtagaacatgaaataacaatataattatcgtatgagttaaatcttaaaagtcacgtaaaagataatcatgcgtcattttgactcacgcggtcgttatagttcaaaatcagtgacacttaccgcattgacaagcacgcctcacgggagctccaagcggcgactgagatgtcctaaatgcacagcgacggattcgcgctatttagaaagagagagcaatatttcaagaatgcatgcgtcaattttacgcagactatctttctagggttaaatcgatagatgcgatcctgcaggtctccctatagtgagtcgtattaatttcgataagccagctgcattaatgaatcggccaacgcgcggggagaggcggtttgcgtattgggcgctcttccgcttcctcgctcactgactcgctgcgctcggtcgttcggctgcggcgagcggtatcagctcactcaaaggcggtaatacggttatccacagaatcaggggataacgcaggaaagaacatgtgagcaaaaggccagcaaaaggccaggaaccgtaaaaaggccgcgttgctggcgtttttccataggctccgcccccctgacgagcatcacaaaaatcgacgctcaagtcagaggtggcgaaacccgacaggactataaagataccaggcgtttccccctggaagctccctcgtgcgctctcctgttccgaccctgccgcttaccggatacctgtccgcctttctcccttcgggaagcgtggcgctttctcatagctcacgctgtaggtatctcagttcggtgtaggtcgttcgctccaagctgggctgtgtgcacgaaccccccgttcagcccgaccgctgcgccttatccggtaactatcgtcttgagtccaacccggtaagacacgacttatcgccactggcagcagccactggtaacaggattagcagagcgaggtatgtaggcggtgctacagagttcttgaagtggtggcctaactacggctacactagaaggacagtatttggtatctgcgctctgctgaagccagttaccttcggaaaaagagttggtagctcttgatccggcaaacaaaccaccgctggtagcggtggtttttttgtttgcaagcagcagattacgcgcagaaaaaaaggatctcaagaagatcctttgatcttttctacggggtctgacgctcagtggaacgaaaactcacgttaagggattttggtcatgagattatcaaaaaggatcttcacctagatccttttaaattaaaaatgaagttttaaatcaatctaaagtatatatgagtaaacttggtctgacagttaccaatgcttaatcagtgaggcacctatctcagcgatctgtctatttcgttcatccatagttgcctgactccccgtcgtgtagataactacgatacgggagggcttaccatctggccccagtgctgcaatgataccgcgagacccacgctcaccggctccagatttatcagcaataaaccagccagccggaagggccgagcgcagaagtggtcctgcaactttatccgcctccatccagtctattaattgttgccgggaagctagagtaagtagttcgccagttaatagtttgcgcaacgttgttgccattgctacaggcatcgtggtgtcacgctcgtcgtttggtatggcttcattcagctccggttcccaacgatcaaggcgagttacatgatcccccatgttgtgcaaaaaagcggttagctccttcggtcctccgatcgttgtcagaagtaagttggccgcagtgttatcactcatggttatggcagcactgcataattctcttactgtcatgccatccgtaagatgcttttctgtgactggtgagtactcaaccaagtcattctgagaatagtgtatgcggcgaccgagttgctcttgcccggcgtcaatacgggataataccgcgccacatagcagaactttaaaagtgctcatcattggaaaacgttcttcggggcgaaaactctcaaggatcttaccgctgttgagatccagttcgatgtaacccactcgtgcacccaactgatcttcagcatcttttactttcaccagcgtttctgggtgagcaaaaacaggaaggcaaaatgccgcaaaaaagggaataagggcgacacggaaatgttgaatactcatactcttcctttttcaatattattgaagcatttatcagggttattgtctcatgagcggatacatatttgaatgtatttagaaaaataaacaaataggggttccgcgcacatttccccgaaaagtgccacctgacgtctaagaaaccattattatcatgacattaacctataaaaataggcgtatcacgaggccctttcgtctcgcgcgtttcggtgatgacggtgaaaacctctgacacatgcagctcccggagacggtcacagcttgtctgtaagcggatgccgggagcagacaagcccgtcagggcgcgtcagcgggtgttggcgggtgtcggggctggcttaactatgcggcatcagagcagattgtactgagagtgcaccatatcgacgctctcccttatgcgactcctgcattaggaagcagcccagtagtaggttgaggccgttgagcaccgccgccgcaaggaatggtgcatgcaaggagatggcgcccaacagtcccccggccacggggcctgccaccatacccacgccgaaacaagcgctcatgagcccgaagtggcgagcccgatcttccccatcggtgatgtcggcgatataggcgccagcaaccgcacctgtggcgccggtgatgccggccacgatgcgtccggcgtagaggatctggctagcgatgaccctgctgattggttcgctgaccatttccggggtgcggaacggcgttaccagaaactcagaaggttcgtccaaccaaaccgactctgacggcagtttacgagagagatgatagggtctgcttcagtaagccagatgctacacaattaggcttgtacatattgtcgttagaacgcggctacaattaatacataaccttatgtatcatacacatacgatttaggtgacactatagaatacacctgcaggacgtcccaatgatcttaagttaa

SEQ ID NO: 28 - DNA, 10755 bp, Artificial Sequence
  pCLD16
ccctagaaagataatcatattgtgacgtacgttaaagataatcatgcgtaaaattgacgcatgtgttttatcggtctgtatatcgaggtttatttattaatttgaatagatattaagttttattatatttacacttacatactaataataaattcaacaaacaatttatttatgtttatttatttattaaaaaaaaacaaaaactcaaaatttcttctataaagtaacaaaacttttatcgaatttgcagcccgggactagctagagggacagcccccccccaaagcccccagggatgtaattacgtccctcccccgctagggggcagcagcgagccgcccggggctccgctccggtccggcgctccccccgcatccccgagccggcagcgtgcggggacagcccgggcacggggaaggtggcacgggatcgctttcctctgaacgcttctcgctgctctttgagcctgcagacacctggggggatacggggaaaacttaagatccgaccggacgcgtactgagagcgctattctgaacttttcttttgttcccttcccttctaccacaccctaattgtaatccattttaatttcctggtcacagtcctgtctctccttccattgtaccttgcccttttctaaagagcgactgcaaagtatgtttgcgtaggtgaggatctaaaactttatgaggtacgaacatcacagaattactttgtaatttcagtttattgtaggcttggctttttggggagggtttacgtcttagacctcttagtgcttctttgtttcatggtgttctaacttcgaagcatctctgtagctttaatggattccttttctgaaagctttgctctctttcttccccctcggctttctcttaggcaagagggctaactgtaaagtaaggcttactgccttgtgtttccaaatgtgtccgaagaggaagtgtcttctgtgaatcctgttatgcatgaataacaggaaatagaaagaaattcactttcattattataaaagtaatatgttcgtttaaaaaattctaatgaagagctggagatgcaacccaggggtagagcacacactcagcatgcaggaggccctgggtccaatcttggaatctcctctcagttaacctgatctctagctgattagtagtgagtgcaagcccactttcctcttctgcctcattgctcagtgataacagctgttaaactttgtcttattctaaaactacctctgtgcaaatgctagcacaataatatatatcatatgcacatgattttttttttatcttgaaaagtaagtcagtatagctacaaagttcacttggcattgtcaacatttcacaggcgtaatattcctcctctagtactgtcctcttcattctttgtgaccaagtttggagagagtgcacaaatgccagggaggtttgtgggaaggtttctcatgttctggtaaggcgagtaagaaaatagtctcatgcaggtgaaatgagtgctatgcagtatatattataccagagaacagcaaatgaccaaattcacactgaactagttcagtaaaattggctttgtcaaagctttccttgcttaaaatgtaattccctgtcatcctagttctggtctggattcttttcctggagtcttgacttccagattccctgtggacttttgtttgagtttcaagcttttgaaatatagaaacctatctaacttaacaaacttgggagagaaaagactccagaacaactgaaaacagaccaggctaaatgaatagactttattcctctcttcttacctgcagttttcagatatgcagagttggagcggatcttagaggttgattcattcatgcctgaagaaaacacattttatagaccctgtgcccaagttcgtggtggacatcaccctttatttactaattgcactacataacaggcattttagaagactgctccagtcagagaccccgccttagaggaatctgtaaaccctgaactcctatcactcatgagcactagttatgtttggaatgccgtattaaaacaaaagttacatttctaaacttaaaattttctagcacagagacagtgggagtagctaactttgatagacatttttctactaaaagtctttctaagtacataatcttctgtaagttggaaaacagcaaaatagaacgtctcctacgtagttaatctttttgcataatttgcacatgtaggagttattagtatacgggtaagttttcactttttcccccaactggagtgtcttgtggctgggtttgaaaaagggaacgggaggccgctggaggggattggtaaatgagataaaacaccactcattcaactcagtgactcagcatttaaattttccataaaaggattaaaggaaaattaaacaaattcttaaagccaagactctggagaaacttgttggtgtgctttagttttcactgttatgactcatgaatttatgcataaattagtacatttataaaaacatagcctttttagagttttctgtttggctaaagtgccattgttagcatttggaattacctttttatgtcttatattttttccaaataaaaataaatgtttctgctgtcttactactgaaactacgttgtgagcactttaaatttctcaaagcagtttcgcctgttatacttggcgcttagtcatcgtcgtacacaacaggacctgattaagaaggctgtgctgcctctaagccgggctagattgtagccactagcaaccaggctgcaataatttccctttgatgacatcatccactgtggaagaacccagttgcttcagccagtcgaactatacagttccaacctcatcaaatatggcatctcccttgcctgctatagcagggggaggaaaaaatgccaccatctttttaatctagcaagcttctcttttcttcatctttttttttttcttttaaaaaaattctgatcatggatgcttcttccgatccctatttgccttatgacgggggaggagacaatatccccttgagggaattacataaaagaggtaagagcatccccttgctctgaatcctctgttggttgttgtgcatgcggctgggcggttctggggacaggctgtctgttgtcctcttgctgcaatgtgctgcttagttgccctgccttgttgctgtgggagaatgcgaccttcccagcagggctggccctccctgattgtttgctctgtgcagattagccctgcttcagatcacatagggctgcagactccatcttctgtgtgaaaatgctttcggtttgattgcagaaataagctgcctttacagccagctaaagtcctggtggttggttggcacctgcaaagtagtatttttgtacctctggaaacttatattttctttacacagcaatatcaagtgccggtatgccattctgttttggctgctgccaattaccatgtagactttgcaccacagagtaatagtaaaagctcctagctgcattttataacatttaaaaatagcaggaaagaagaattatttttgatttaacatgtttttgtcatttaacgtcttaactgattgacatactatattgtctgtctcgtgggtatcttgtacaacttgataggataaagcaatttagtttttttttttttttttaaatacatccagaatgtaagtcgtcagtagttttcgaacagataagtaatggtgttaatcttttggcaggctttgccttggtctccttaaagctaattaggtgttacttaattaaactgctcttttgctcattttcttaaattatttttttaaaagatagttggcatttgctgttctagaaataaacttcaagaaacattctttagccagatgacttcatgtatgagccatgttagtttgaattatttgcttggtgttataaactttatggtttaataccaacttttattatgtttacaaggtaaataaggaaaatttcaagtacattttgtatcctgagaacaaatttaagttccatagaatttaggaattacaatgtattcaacagatacttacttgtcatactgtgcctgcaaaacaataattagactctgaacaggtgcaacaattttctgtagaattagacaagtcttcttttggcaggtgttactaagtaggccatttcccaaggaacagggaatttgccaggcttttgtggtggagagaatagaatgaataaatgctgtggggagtaaagagcttgtcagaagatgattagttctgtggcaccaaaaccaagagatcagttttcctgtgagaagtaaaggaagcattgtagaaaaatagatgtgttgaagtctaccggtggagttccgcgttacataacttacggtaaatggcccgcctggctgaccgcccaacgacccccgcccattgacgtcaataatgacgtatgttcccatagtaacgccaatagggactttccattgacgtcaatgggtggagtatttacggtaaactgcccacttggcagtacatcaagtgtatcatatgccaagtacgccccctattgacgtcaatgacggtaaatggcccgcctggcattatgcccagtacatgaccttatgggactttcctacttggcagtacatctacgtattagtcatcgctattaccattgtgatgcggttttggcagtacatcaatgggcgtggatagcggtttgactcacggggatttccaagtctccaccccattgacgtcaatgggagtttgttttggcaccaaaatcaacgggactttccaaaatgtcgtaacaactccgccccattgacgcaaatgggcggtaggcgtgtacggtgggaggtctatataagcagagctcgtttagtgaaccgtcagatctacctcttccgcatcgctgtctgcgagggccagctgttggggtgagtactccctctcaaaagcgggcatgacttctgcgctaagattgtcagtttccaaaaacgaggaggatttgatattcacctggcccgcggtgatgcctttgagggtggccgcgtccatctggtcagaaaagacaatctttttgttgtcaagcttccttgatgatgtcatacttatcctgtcccttttttttccacagctcgcggttgaggacaaactcttcgcggtctttccagtactcttggatcggaaacccgtcggcctccgaacggtactccgccaccgagggacctgagcgagtccgcatcgaccggatcggaaaacctcggatccgaattcatagataactgatccagtgcccctaacgttactggccgaagccgcttggaataaggccggtgtgcgtttgtctatatgttattttccaccatattgccgtcttttggcaatgtgagggcccggaaacctggccctgtcttcttgacgagcattcctaggggtctttcccctctcgccaaaggaatgcaaggtctgttgaatgtcgtgaaggaagcagttcctctggaagcttcttgaagacaaacaacgtctgtagcgaccctttgcaggcagcggaaccccccacctggcgacaggtgcctctgcggccaaaagccacgtgtataagatacacctgcaaaggcggcacaaccccagtgccacgttgtgagttggatagttgtggaaagagtcaaatggctctcctcaagcgtattcaacaaggggctgaaggatgcccagaaggtaccccattgtatgggatctgatctggggcctcggtgcacatgctttacatgtgtttagtcgaggttaaaaaaacgtctaggccccccgaaccacggggacgtggttttcctttgaaaaacacgatgataaatggccacctcagcaagttcccacttgaacaaaaacatcaagcaaatgtacttgtgcctgccccagggtgagaaagtccaagccatgtatatctgggttgatggtactggagaaggactgcgctgcaaaacccgcaccctggactgtgagcccaagtgtgtagaagagttacctgagtggaattttgatggctctagtacctttcagtctgagggctccaacagtgacatgtatctcagccctgttgccatgtttcgggaccccttccgcagagatcccaacaagctggtgttctgtgaagttttcaagtacaaccggaagcctgcagagaccaatttaaggcactcgtgtaaacggataatggacatggtgagcaaccagcacccctggtttggaatggaacaggagtatactctgatgggaacagatgggcacccttttggttggccttccaatggctttcctgggccccaaggtccgtattactgtggtgtgggcgcagacaaagcctatggcagggatatcgtggaggctcactaccgcgcctgcttgtatgctggggtcaagattacaggaacaaatgctgaggtcatgcctgcccagtgggagttccaaataggaccctgtgaaggaatccgcatgggagatcatctctgggtggcccgtttcatcttgcatcgagtatgtgaagactttggggtaatagcaacctttgaccccaagcccattcctgggaactggaatggtgcaggctgccataccaactttagcaccaaggccatgcgggaggagaatggtctgaagcacatcgaggaggccatcgagaaactaagcaagcggcaccggtaccacattcgagcctacgatcccaaggggggcctggacaatgcccgtcgtctgactgggttccacgaaacgtccaacatcaacgacttttctgctggtgtcgccaatcgcagtgccagcatccgcattccccggactgtcggccaggagaagaaaggttactttgaagaccgccgcccctctgccaattgtgacccctttgcagtgacagaagccatcgtccgcacatgccttctcaatgagactggcgacgagcccttccaatacaaaaactaatctagatccccctcgctttcttgctgtccaatttctattaaaggttcctttgttccctaagtccaactactaaactgggggatattatgaagggccttgagcatctggattctgcctaataaaaaacatttattttcattgcaatgatgtatttaaattatttctgaatattttactaaaaagggaatgtgggaggtcagtgcatttaaaacataaagaaatgaagagggggatcttcgcgatactgcatcgatgagggacagcccccccccaaagcccccagggatgtaattacgtccctcccccgctagggggcagcagcgagccgcccggggctccgctccggtccggcgctccccccgcatccccgagccggcagcgtgcggggacagcccgggcacggggaaggtggcacgggatcgctttcctctgaacgcttctcgctgctctttgagcctgcagacacctggggggatacggggaaaatagacaccgcggtggagctccagcttttgttccctttagtgagggttaattagttcttaatacgactcactatagggcgaattggctaccgggccgcccatcgagggtatcataagcttatatctataacaagaaaatatatatataataagttatcacgtaagtagaacatgaaataacaatataattatcgtatgagttaaatcttaaaagtcacgtaaaagataatcatgcgtcattttgactcacgcggtcgttatagttcaaaatcagtgacacttaccgcattgacaagcacgcctcacgggagctccaagcggcgactgagatgtcctaaatgcacagcgacggattcgcgctatttagaaagagagagcaatatttcaagaatgcatgcgtcaattttacgcagactatctttctagggttaaatcgatagatgcgatcctgcaggtctccctatagtgagtcgtattaatttcgataagccagctgcattaatgaatcggccaacgcgcggggagaggcggtttgcgtattgggcgctcttccgcttcctcgctcactgactcgctgcgctcggtcgttcggctgcggcgagcggtatcagctcactcaaaggcggtaatacggttatccacagaatcaggggataacgcaggaaagaacatgtgagcaaaaggccagcaaaaggccaggaaccgtaaaaaggccgcgttgctggcgtttttccataggctccgcccccctgacgagcatcacaaaaatcgacgctcaagtcagaggtggcgaaacccgacaggactataaagataccaggcgtttccccctggaagctccctcgtgcgctctcctgttccgaccctgccgcttaccggatacctgtccgcctttctcccttcgggaagcgtggcgctttctcatagctcacgctgtaggtatctcagttcggtgtaggtcgttcgctccaagctgggctgtgtgcacgaaccccccgttcagcccgaccgctgcgccttatccggtaactatcgtcttgagtccaacccggtaagacacgacttatcgccactggcagcagccactggtaacaggattagcagagcgaggtatgtaggcggtgctacagagttcttgaagtggtggcctaactacggctacactagaaggacagtatttggtatctgcgctctgctgaagccagttaccttcggaaaaagagttggtagctcttgatccggcaaacaaaccaccgctggtagcggtggtttttttgtttgcaagcagcagattacgcgcagaaaaaaaggatctcaagaagatcctttgatcttttctacggggtctgacgctcagtggaacgaaaactcacgttaagggattttggtcatgagattatcaaaaaggatcttcacctagatccttttaaattaaaaatgaagttttaaatcaatctaaagtatatatgagtaaacttggtctgacagttaccaatgcttaatcagtgaggcacctatctcagcgatctgtctatttcgttcatccatagttgcctgactccccgtcgtgtagataactacgatacgggagggcttaccatctggccccagtgctgcaatgataccgcgagacccacgctcaccggctccagatttatcagcaataaaccagccagccggaagggccgagcgcagaagtggtcctgcaactttatccgcctccatccagtctattaattgttgccgggaagctagagtaagtagttcgccagttaatagtttgcgcaacgttgttgccattgctacaggcatcgtggtgtcacgctcgtcgtttggtatggcttcattcagctccggttcccaacgatcaaggcgagttacatgatcccccatgttgtgcaaaaaagcggttagctccttcggtcctccgatcgttgtcagaagtaagttggccgcagtgttatcactcatggttatggcagcactgcataattctcttactgtcatgccatccgtaagatgcttttctgtgactggtgagtactcaaccaagtcattctgagaatagtgtatgcggcgaccgagttgctcttgcccggcgtcaatacgggataataccgcgccacatagcagaactttaaaagtgctcatcattggaaaacgttcttcggggcgaaaactctcaaggatcttaccgctgttgagatccagttcgatgtaacccactcgtgcacccaactgatcttcagcatcttttactttcaccagcgtttctgggtgagcaaaaacaggaaggcaaaatgccgcaaaaaagggaataagggcgacacggaaatgttgaatactcatactcttcctttttcaatattattgaagcatttatcagggttattgtctcatgagcggatacatatttgaatgtatttagaaaaataaacaaataggggttccgcgcacatttccccgaaaagtgccacctgacgtctaagaaaccattattatcatgacattaacctataaaaataggcgtatcacgaggccctttcgtctcgcgcgtttcggtgatgacggtgaaaacctctgacacatgcagctcccggagacggtcacagcttgtctgtaagcggatgccgggagcagacaagcccgtcagggcgcgtcagcgggtgttggcgggtgtcggggctggcttaactatgcggcatcagagcagattgtactgagagtgcaccatatcgacgctctcccttatgcgactcctgcattaggaagcagcccagtagtaggttgaggccgttgagcaccgccgccgcaaggaatggtgcatgcaaggagatggcgcccaacagtcccccggccacggggcctgccaccatacccacgccgaaacaagcgctcatgagcccgaagtggcgagcccgatcttccccatcggtgatgtcggcgatataggcgccagcaaccgcacctgtggcgccggtgatgccggccacgatgcgtccggcgtagaggatctggctagcgatgaccctgctgattggttcgctgaccatttccggggtgcggaacggcgttaccagaaactcagaaggttcgtccaaccaaaccgactctgacggcagtttacgagagagatgatagggtctgcttcagtaagccagatgctacacaattaggcttgtacatattgtcgttagaacgcggctacaattaatacataaccttatgtatcatacacatacgatttaggtgacactatagaatacacctgcaggacgtcccaatgatcttaagttaa

SEQ ID NO: 29 - DNA, 10748 bp, Artificial Sequence
  pCLD17
ccctagaaagataatcatattgtgacgtacgttaaagataatcatgcgtaaaattgacgcatgtgttttatcggtctgtatatcgaggtttatttattaatttgaatagatattaagttttattatatttacacttacatactaataataaattcaacaaacaatttatttatgtttatttatttattaaaaaaaaacaaaaactcaaaatttcttctataaagtaacaaaacttttatcgaatttgcagcccgggactagctagagggacagcccccccccaaagcccccagggatgtaattacgtccctcccccgctagggggcagcagcgagccgcccggggctccgctccggtccggcgctccccccgcatccccgagccggcagcgtgcggggacagcccgggcacggggaaggtggcacgggatcgctttcctctgaacgcttctcgctgctctttgagcctgcagacacctggggggatacggggaaaacttaagatccgaccggacgcgtactgagagcgctattctgaacttttcttttgttcccttcccttctaccacaccctaattgtaatccattttaatttcctggtcacagtcctgtctctccttccattgtaccttgcccttttctaaagagcgactgcaaagtatgtttgcgtaggtgaggatctaaaactttatgaggtacgaacatcacagaattactttgtaatttcagtttattgtaggcttggctttttggggagggtttacgtcttagacctcttagtgcttctttgtttcatggtgttctaacttcgaagcatctctgtagctttaatggattccttttctgaaagctttgctctctttcttccccctcggctttctcttaggcaagagggctaactgtaaagtaaggcttactgccttgtgtttccaaatgtgtccgaagaggaagtgtcttctgtgaatcctgttatgcatgaataacaggaaatagaaagaaattcactttcattattataaaagtaatatgttcgtttaaaaaattctaatgaagagctggagatgcaacccaggggtagagcacacactcagcatgcaggaggccctgggtccaatcttggaatctcctctcagttaacctgatctctagctgattagtagtgagtgcaagcccactttcctcttctgcctcattgctcagtgataacagctgttaaactttgtcttattctaaaactacctctgtgcaaatgctagcacaataatatatatcatatgcacatgattttttttttatcttgaaaagtaagtcagtatagctacaaagttcacttggcattgtcaacatttcacaggcgtaatattcctcctctagtactgtcctcttcattctttgtgaccaagtttggagagagtgcacaaatgccagggaggtttgtgggaaggtttctcatgttctggtaaggcgagtaagaaaatagtctcatgcaggtgaaatgagtgctatgcagtatatattataccagagaacagcaaatgaccaaattcacactgaactagttcagtaaaattggctttgtcaaagctttccttgcttaaaatgtaattccctgtcatcctagttctggtctggattcttttcctggagtcttgacttccagattccctgtggacttttgtttgagtttcaagcttttgaaatatagaaacctatctaacttaacaaacttgggagagaaaagactccagaacaactgaaaacagaccaggctaaatgaatagactttattcctctcttcttacctgcagttttcagatatgcagagttggagcggatcttagaggttgattcattcatgcctgaagaaaacacattttatagaccctgtgcccaagttcgtggtggacatcaccctttatttactaattgcactacataacaggcattttagaagactgctccagtcagagaccccgccttagaggaatctgtaaaccctgaactcctatcactcatgagcactagttatgtttggaatgccgtattaaaacaaaagttacatttctaaacttaaaattttctagcacagagacagtgggagtagctaactttgatagacatttttctactaaaagtctttctaagtacataatcttctgtaagttggaaaacagcaaaatagaacgtctcctacgtagttaatctttttgcataatttgcacatgtaggagttattagtatacgggtaagttttcactttttcccccaactggagtgtcttgtggctgggtttgaaaaagggaacgggaggccgctggaggggattggtaaatgagataaaacaccactcattcaactcagtgactcagcatttaaattttccataaaaggattaaaggaaaattaaacaaattcttaaagccaagactctggagaaacttgttggtgtgctttagttttcactgttatgactcatgaatttatgcataaattagtacatttataaaaacatagcctttttagagttttctgtttggctaaagtgccattgttagcatttggaattacctttttatgtcttatattttttccaaataaaaataaatgtttctgctgtcttactactgaaactacgttgtgagcactttaaatttctcaaagcagtttcgcctgttatacttggcgcttagtcatcgtcgtacacaacaggacctgattaagaaggctgtgctgcctctaagccgggctagattgtagccactagcaaccaggctgcaataatttccctttgatgacatcatccactgtggaagaacccagttgcttcagccagtcgaactatacagttccaacctcatcaaatatggcatctcccttgcctgctatagcagggggaggaaaaaatgccaccatctttttaatctagcaagcttctcttttcttcatctttttttttttcttttaaaaaaattctgatcatggatgcttcttccgatccctatttgccttatgacgggggaggagacaatatccccttgagggaattacataaaagaggtaagagcatccccttgctctgaatcctctgttggttgttgtgcatgcggctgggcggttctggggacaggctgtctgttgtcctcttgctgcaatgtgctgcttagttgccctgccttgttgctgtgggagaatgcgaccttcccagcagggctggccctccctgattgtttgctctgtgcagattagccctgcttcagatcacatagggctgcagactccatcttctgtgtgaaaatgctttcggtttgattgcagaaataagctgcctttacagccagctaaagtcctggtggttggttggcacctgcaaagtagtatttttgtacctctggaaacttatattttctttacacagcaatatcaagtgccggtatgccattctgttttggctgctgccaattaccatgtagactttgcaccacagagtaatagtaaaagctcctagctgcattttataacatttaaaaatagcaggaaagaagaattatttttgatttaacatgtttttgtcatttaacgtcttaactgattgacatactatattgtctgtctcgtgggtatcttgtacaacttgataggataaagcaatttagtttttttttttttttttaaatacatccagaatgtaagtcgtcagtagttttcgaacagataagtaatggtgttaatcttttggcaggctttgccttggtctccttaaagctaattaggtgttacttaattaaactgctcttttgctcattttcttaaattatttttttaaaagatagttggcatttgctgttctagaaataaacttcaagaaacattctttagccagatgacttcatgtatgagccatgttagtttgaattatttgcttggtgttataaactttatggtttaataccaacttttattatgtttacaaggtaaataaggaaaatttcaagtacattttgtatcctgagaacaaatttaagttccatagaatttaggaattacaatgtattcaacagatacttacttgtcatactgtgcctgcaaaacaataattagactctgaacaggtgcaacaattttctgtagaattagacaagtcttcttttggcaggtgttactaagtaggccatttcccaaggaacagggaatttgccaggcttttgtggtggagagaatagaatgaataaatgctgtggggagtaaagagcttgtcagaagatgattagttctgtggcaccaaaaccaagagatcagttttcctgtgagaagtaaaggaagcattgtagaaaaatagatgtgttgaagtctaccggtggagttccgcgttacataacttacggtaaatggcccgcctggctgaccgcccaacgacccccgcccattgacgtcaataatgacgtatgttcccatagtaacgccaatagggactttccattgacgtcaatgggtggagtatttacggtaaactgcccacttggcagtacatcaagtgtatcatatgccaagtacgccccctattgacgtcaatgacggtaaatggcccgcctggcattatgcccagtacatgaccttatgggactttcctacttggcagtacatctacgtattagtcatcgctattaccattgtgatgcggttttggcagtacatcaatgggcgtggatagcggtttgactcacggggatttccaagtctccaccccattgacgtcaatgggagtttgttttggcaccaaaatcaacgggactttccaaaatgtcgtaacaactccgccccattgacgcaaatgggcggtaggcgtgtacggtgggaggtctatataagcagagctcgtttagtgaaccgtcagatctacctcttccgcatcgctgtctgcgagggccagctgttggggtgagtactccctctcaaaagcgggcatgacttctgcgctaagattgtcagtttccaaaaacgaggaggatttgatattcacctggcccgcggtgatgcctttgagggtggccgcgtccatctggtcagaaaagacaatctttttgttgtcaagcttccttgatgatgtcatacttatcctgtcccttttttttccacagctcgcggttgaggacaaactcttcgcggtctttccagtactcttggatcggaaacccgtcggcctccgaacggtactccgccaccgagggacctgagcgagtccgcatcgaccggatcggaaaacctcggatccgaattcatagataactgatccagtgcccctaacgttactggccgaagccgcttggaataaggccggtgtgcgtttgtctatatgttattttccaccatattgccgtcttttggcaatgtgagggcccggaaacctggccctgtcttcttgacgagcattcctaggggtctttcccctctcgccaaaggaatgcaaggtctgttgaatgtcgtgaaggaagcagttcctctggaagcttcttgaagacaaacaacgtctgtagcgaccctttgcaggcagcggaaccccccacctggcgacaggtgcctctgcggccaaaagccacgtgtataagatacacctgcaaaggcggcacaaccccagtgccacgttgtgagttggatagttgtggaaagagtcaaatggctctcctcaagcgtattcaacaaggggctgaaggatgcccagaaggtaccccattgtatgggatctgatctggggcctcggtgcacatgctttacatgtgtttagtcgaggttaaaaaaacgtctaggccccccgaaccacggggacgtggttttcctttgaaaaacacgatggccacctcagcaagttcccacttgaacaaaaacatcaagcaaatgtacttgtgcctgccccagggtgagaaagtccaagccatgtatatctgggttgatggtactggagaaggactgcgctgcaaaacccgcaccctggactgtgagcccaagtgtgtagaagagttacctgagtggaattttgatggctctagtacctttcagtctgagggctccaacagtgacatgtatctcagccctgttgccatgtttcgggaccccttccgcagagatcccaacaagctggtgttctgtgaagttttcaagtacaaccggaagcctgcagagaccaatttaaggcactcgtgtaaacggataatggacatggtgagcaaccagcacccctggtttggaatggaacaggagtatactctgatgggaacagatgggcacccttttggttggccttccaatggctttcctgggccccaaggtccgtattactgtggtgtgggcgcagacaaagcctatggcagggatatcgtggaggctcactaccgcgcctgcttgtatgctggggtcaagattacaggaacaaatgctgaggtcatgcctgcccagtgggagttccaaataggaccctgtgaaggaatccgcatgggagatcatctctgggtggcccgtttcatcttgcatcgagtatgtgaagactttggggtaatagcaacctttgaccccaagcccattcctgggaactggaatggtgcaggctgccataccaactttagcaccaaggccatgcgggaggagaatggtctgaagcacatcgaggaggccatcgagaaactaagcaagcggcaccggtaccacattcgagcctacgatcccaaggggggcctggacaatgcccgtcgtctgactgggttccacgaaacgtccaacatcaacgacttttctgctggtgtcgccaatcgcagtgccagcatccgcattccccggactgtcggccaggagaagaaaggttactttgaagaccgccgcccctctgccaattgtgacccctttgcagtgacagaagccatcgtccgcacatgccttctcaatgagactggcgacgagcccttccaatacaaaaactaatctagatccccctcgctttcttgctgtccaatttctattaaaggttcctttgttccctaagtccaactactaaactgggggatattatgaagggccttgagcatctggattctgcctaataaaaaacatttattttcattgcaatgatgtatttaaattatttctgaatattttactaaaaagggaatgtgggaggtcagtgcatttaaaacataaagaaatgaagagggggatcttcgcgatactgcatcgatgagggacagcccccccccaaagcccccagggatgtaattacgtccctcccccgctagggggcagcagcgagccgcccggggctccgctccggtccggcgctccccccgcatccccgagccggcagcgtgcggggacagcccgggcacggggaaggtggcacgggatcgctttcctctgaacgcttctcgctgctctttgagcctgcagacacctggggggatacggggaaaatagacaccgcggtggagctccagcttttgttccctttagtgagggttaattagttcttaatacgactcactatagggcgaattggctaccgggccgcccatcgagggtatcataagcttatatctataacaagaaaatatatatataataagttatcacgtaagtagaacatgaaataacaatataattatcgtatgagttaaatcttaaaagtcacgtaaaagataatcatgcgtcattttgactcacgcggtcgttatagttcaaaatcagtgacacttaccgcattgacaagcacgcctcacgggagctccaagcggcgactgagatgtcctaaatgcacagcgacggattcgcgctatttagaaagagagagcaatatttcaagaatgcatgcgtcaattttacgcagactatctttctagggttaaatcgatagatgcgatcctgcaggtctccctatagtgagtcgtattaatttcgataagccagctgcattaatgaatcggccaacgcgcggggagaggcggtttgcgtattgggcgctcttccgcttcctcgctcactgactcgctgcgctcggtcgttcggctgcggcgagcggtatcagctcactcaaaggcggtaatacggttatccacagaatcaggggataacgcaggaaagaacatgtgagcaaaaggccagcaaaaggccaggaaccgtaaaaaggccgcgttgctggcgtttttccataggctccgcccccctgacgagcatcacaaaaatcgacgctcaagtcagaggtggcgaaacccgacaggactataaagataccaggcgtttccccctggaagctccctcgtgcgctctcctgttccgaccctgccgcttaccggatacctgtccgcctttctcccttcgggaagcgtggcgctttctcatagctcacgctgtaggtatctcagttcggtgtaggtcgttcgctccaagctgggctgtgtgcacgaaccccccgttcagcccgaccgctgcgccttatccggtaactatcgtcttgagtccaacccggtaagacacgacttatcgccactggcagcagccactggtaacaggattagcagagcgaggtatgtaggcggtgctacagagttcttgaagtggtggcctaactacggctacactagaaggacagtatttggtatctgcgctctgctgaagccagttaccttcggaaaaagagttggtagctcttgatccggcaaacaaaccaccgctggtagcggtggtttttttgtttgcaagcagcagattacgcgcagaaaaaaaggatctcaagaagatcctttgatcttttctacggggtctgacgctcagtggaacgaaaactcacgttaagggattttggtcatgagattatcaaaaaggatcttcacctagatccttttaaattaaaaatgaagttttaaatcaatctaaagtatatatgagtaaacttggtctgacagttaccaatgcttaatcagtgaggcacctatctcagcgatctgtctatttcgttcatccatagttgcctgactccccgtcgtgtagataactacgatacgggagggcttaccatctggccccagtgctgcaatgataccgcgagacccacgctcaccggctccagatttatcagcaataaaccagccagccggaagggccgagcgcagaagtggtcctgcaactttatccgcctccatccagtctattaattgttgccgggaagctagagtaagtagttcgccagttaatagtttgcgcaacgttgttgccattgctacaggcatcgtggtgtcacgctcgtcgtttggtatggcttcattcagctccggttcccaacgatcaaggcgagttacatgatcccccatgttgtgcaaaaaagcggttagctccttcggtcctccgatcgttgtcagaagtaagttggccgcagtgttatcactcatggttatggcagcactgcataattctcttactgtcatgccatccgtaagatgcttttctgtgactggtgagtactcaaccaagtcattctgagaatagtgtatgcggcgaccgagttgctcttgcccggcgtcaatacgggataataccgcgccacatagcagaactttaaaagtgctcatcattggaaaacgttcttcggggcgaaaactctcaaggatcttaccgctgttgagatccagttcgatgtaacccactcgtgcacccaactgatcttcagcatcttttactttcaccagcgtttctgggtgagcaaaaacaggaaggcaaaatgccgcaaaaaagggaataagggcgacacggaaatgttgaatactcatactcttcctttttcaatattattgaagcatttatcagggttattgtctcatgagcggatacatatttgaatgtatttagaaaaataaacaaataggggttccgcgcacatttccccgaaaagtgccacctgacgtctaagaaaccattattatcatgacattaacctataaaaataggcgtatcacgaggccctttcgtctcgcgcgtttcggtgatgacggtgaaaacctctgacacatgcagctcccggagacggtcacagcttgtctgtaagcggatgccgggagcagacaagcccgtcagggcgcgtcagcgggtgttggcgggtgtcggggctggcttaactatgcggcatcagagcagattgtactgagagtgcaccatatcgacgctctcccttatgcgactcctgcattaggaagcagcccagtagtaggttgaggccgttgagcaccgccgccgcaaggaatggtgcatgcaaggagatggcgcccaacagtcccccggccacggggcctgccaccatacccacgccgaaacaagcgctcatgagcccgaagtggcgagcccgatcttccccatcggtgatgtcggcgatataggcgccagcaaccgcacctgtggcgccggtgatgccggccacgatgcgtccggcgtagaggatctggctagcgatgaccctgctgattggttcgctgaccatttccggggtgcggaacggcgttaccagaaactcagaaggttcgtccaaccaaaccgactctgacggcagtttacgagagagatgatagggtctgcttcagtaagccagatgctacacaattaggcttgtacatattgtcgttagaacgcggctacaattaatacataaccttatgtatcatacacatacgatttaggtgacactatagaatacacctgcaggacgtcccaatgatcttaagttaa